European Patent Specification EP 3 596 125 B1, published November 19, 2025. Title: ANTI-PAR2 ANTIBODIES AND USES THEREOF. Applicant: MEDIMMUNE LIMITED. The sequence listing filed with the application follows.

SEQUENCE LISTING (841 sequences)

SEQ ID NO: 1 - DNA, 351 bp, Homo sapiens
gaggtgcagctgctcgagagcggcggagggctggtgcagccaggcggcagcctgaggctgtcctgcgccgcctccggattcaccttcagcagctacgccatgaactgggtgcggcaggccccaggcaagggcctggagtgggtgtccaccatcagctacagcgggtcgctgatcagctacgccgacagcgtgaagggcaggttcaccatcagcagggacaacagcaagaacaccctgtacctgcagatgaacagcctgagggccgaggacaccgccgtgtactactgcgcccgcatcaacaacgaccctatggatgtgtggggccagggcaccctggtgacagtgagctca

SEQ ID NO: 2 - protein, 117 aa, Homo sapiens
EVQLLESGGGLVQPGGSLRLSCAASGFTFSSYAMNWVRQAPGKGLEWVSTISYSGSLISYADSVKGRFTISRDNSKNTLYLQMNSLRAEDTAVYYCARINNDPMDVWGQGTLVTVSS

SEQ ID NO: 3 - protein, 5 aa, Homo sapiens
SYAMN

SEQ ID NO: 4 - protein, 17 aa, Homo sapiens
TISYSGSLISYADSVKG

SEQ ID NO: 5 - protein, 8 aa, Homo sapiens
INNDPMDV

SEQ ID NO: 6 - DNA, 333 bp, Homo sapiens
agtatcgagctgacccagccccccagcgtgagcgtgtccccaggccagaccgccagcatcacctgcagcggcgacaacctgggcaagaaatacgtgcagtggtatcagcagaagcccggccagtcccccgtgctggtgatctacgacgacagcaacaggcccagcggcatccccgagaggttcagcggcagcaacagcggcaacaccgccaccctgaccatcagcggcacccaggccatggacgaggccgactactactgccagacctgggacgggaacccgacgacgggcgagaccaacgtgttcggcggagggaccaagttaaccgtccta

SEQ ID NO: 7 - protein, 111 aa, Homo sapiens
SIELTQPPSVSVSPGQTASITCSGDNLGKKYVQWYQQKPGQSPVLVIYDDSNRPSGIPERFSGSNSGNTATLTISGTQAMDEADYYCQTWDGNPTTGETNVFGGGTKLTVL

SEQ ID NO: 8 - protein, 11 aa, Homo sapiens
SGDNLGKKYVQ

SEQ ID NO: 9 - protein, 7 aa, Homo sapiens
DDSNRPS

SEQ ID NO: 10 - protein, 14 aa, Homo sapiens
QTWDGNPTTGETNV

SEQ ID NO: 11 - DNA, 351 bp, Homo sapiens
gaggtgcagctgctggagagcggcggagggctggtgcagccaggcggcagcctgaggctgtcctgcgccgcctccggattcaccttcagcagctacgccatgaactgggtgcggcaggccccaggcaagggcctggagtgggtgtccaccatcagctaccacgggtcgcacatcagctaccacgacagcgtgcatcacaggttcaccatcagcagggacaacagcaagaacaccctgtacctgcagatgaacagcctgagggccgaggacaccgccgtgtactactgcgcccgcatccaccacgaccctatggatgtgtggggccagggcaccctggtgacagtgagctca

SEQ ID NO: 12 - protein, 117 aa, Homo sapiens
EVQLLESGGGLVQPGGSLRLSCAASGFTFSSYAMNWVRQAPGKGLEWVSTISYHGSHISYHDSVHHRFTISRDNSKNTLYLQMNSLRAEDTAVYYCARIHHDPMDVWGQGTLVTVSS

SEQ ID NO: 13 - protein, 5 aa, Homo sapiens
SYAMN

SEQ ID NO: 14 - protein, 17 aa, Homo sapiens
TISYHGSHISYHDSVHH

SEQ ID NO: 15 - protein, 8 aa, Homo sapiens
IHHDPMDV

SEQ ID NO: 16 - DNA, 333 bp, Homo sapiens
agtatcgagctgacccagccccccagcgtgagcgtgtccccaggccagaccgccagcatcacctgcagcggcgacaacctgggcaagaaatacgtgcagtggtatcagcagaagcccggccagtcccccgtgctggtgatctacgacgacagcaacaggcccagcggcatccccgagaggttcagcggcagcaacagcggcaacaccgccaccctgaccatcagcggcacccaggcgatggacgaggccgactactactgccagacctgggacgggaacccgacgacgggcgagaccaacgtgttcggcggagggaccaagttaaccgtccta

SEQ ID NO: 17 - protein, 111 aa, Homo sapiens; identical to SEQ ID NO: 7

SEQ ID NO: 18 - protein, 11 aa, Homo sapiens
SGDNLGKKYVQ

SEQ ID NO: 19 - protein, 7 aa, Homo sapiens
DDSNRPS

SEQ ID NO: 20 - protein, 14 aa, Homo sapiens
QTWDGNPTTGETNV

SEQ ID NO: 21 - DNA, 351 bp, Homo sapiens
gaggtgcagctgctcgagagcggcggagggctggtgcagccaggcggcagcctgaggctgtcctgcgccgcctccggattcaccttcagcagctacgccatgaactgggtgcggcaggccccaggcaagggcctggagtgggtgtccaccatcagctacagcgggtcgctgatccactacgccgacagcgtgaagggcaggttcaccatcagcagggacaacagcaagaacaccctgtacctgcagatgaacagcctgagggccgaggacaccgccgtgtactactgcgcccgcatcaacaacgaccctatggatgtgtggggccagggcaccctggtgacagtgagctca

SEQ ID NO: 22 - protein, 117 aa, Homo sapiens
EVQLLESGGGLVQPGGSLRLSCAASGFTFSSYAMNWVRQAPGKGLEWVSTISYSGSLIHYADSVKGRFTISRDNSKNTLYLQMNSLRAEDTAVYYCARINNDPMDVWGQGTLVTVSS

SEQ ID NO: 23 - protein, 5 aa, Homo sapiens
SYAMN

SEQ ID NO: 24 - protein, 17 aa, Homo sapiens
TISYSGSLIHYADSVKG

SEQ ID NO: 25 - protein, 8 aa, Homo sapiens
INNDPMDV

SEQ ID NO: 26 - DNA, 333 bp, Homo sapiens; identical to SEQ ID NO: 6

SEQ ID NO: 27 - protein, 111 aa, Homo sapiens; identical to SEQ ID NO: 7

SEQ ID NO: 28 - protein, 11 aa, Homo sapiens
SGDNLGKKYVQ

SEQ ID NO: 29 - protein, 7 aa, Homo sapiens
DDSNRPS

SEQ ID NO: 30 - protein, 14 aa, Homo sapiens
QTWDGNPTTGETNV

SEQ ID NO: 31 - DNA, 351 bp, Homo sapiens
gaggtgcagctgctcgagagcggcggagggctggtgcagccaggcggcagcctgaggctgtcctgcgccgcctccggattcaccttcagcagctacgccatgaactgggtgcggcaggccccaggcaagggcctggagtgggtgtccaccatcagctacagcgggtcgctgatcagctacgccgacagcgtgaagggcaggttcaccatcagcagggacaacagcaagaacaccctgtacctgcagatgaacagcctgagggccgaggacaccgccgtgtactactgcgcccgcatcaaccacgaccctatggatgtgtggggccagggcaccctggtgacagtgagctca

SEQ ID NO: 32 - protein, 117 aa, Homo sapiens
EVQLLESGGGLVQPGGSLRLSCAASGFTFSSYAMNWVRQAPGKGLEWVSTISYSGSLISYADSVKGRFTISRDNSKNTLYLQMNSLRAEDTAVYYCARINHDPMDVWGQGTLVTVSS

SEQ ID NO: 33 - protein, 5 aa, Homo sapiens
SYAMN

SEQ ID NO: 34 - protein, 17 aa, Homo sapiens
TISYSGSLISYADSVKG

SEQ ID NO: 35 - protein, 8 aa, Homo sapiens
INHDPMDV

SEQ ID NO: 36 - DNA, 333 bp, Homo sapiens; identical to SEQ ID NO: 6

SEQ ID NO: 37 - protein, 111 aa, Homo sapiens; identical to SEQ ID NO: 7

SEQ ID NO: 38 - protein, 11 aa, Homo sapiens
SGDNLGKKYVQ

SEQ ID NO: 39 - protein, 7 aa, Homo sapiens
DDSNRPS

SEQ ID NO: 40 - protein, 14 aa, Homo sapiens
QTWDGNPTTGETNV

SEQ ID NO: 41 - DNA, 351 bp, Homo sapiens; identical to SEQ ID NO: 1

SEQ ID NO: 42 - protein, 117 aa, Homo sapiens; identical to SEQ ID NO: 2

SEQ ID NO: 43 - protein, 5 aa, Homo sapiens
SYAMN

SEQ ID NO: 44 - protein, 17 aa, Homo sapiens
TISYSGSLISYADSVKG

SEQ ID NO: 45 - protein, 8 aa, Homo sapiens
INNDPMDV

SEQ ID NO: 46 - DNA, 333 bp, Homo sapiens
agtatcgagctgacccagccccccagcgtgagcgtgtccccaggccagaccgccagcatcacctgcagcggcgacaacctgggcaagaaatacgtgcagtggtatcagcagaagcccggccagtcccccgtgctggtgatctacgacgacagcaacaggcccagcggcatccccgagaggttcagcggcagcaacagcggcaacaccgccaccctgaccatcagcggcacccaggccatggacgaggccgactactactgccagacctgggacgggaacccgacgcacggcgagaccaacgtgttcggcggagggaccaagttaaccgtccta

SEQ ID NO: 47 - protein, 111 aa, Homo sapiens
SIELTQPPSVSVSPGQTASITCSGDNLGKKYVQWYQQKPGQSPVLVIYDDSNRPSGIPERFSGSNSGNTATLTISGTQAMDEADYYCQTWDGNPTHGETNVFGGGTKLTVL

SEQ ID NO: 48 - protein, 11 aa, Homo sapiens
SGDNLGKKYVQ

SEQ ID NO: 49 - protein, 7 aa, Homo sapiens
DDSNRPS

SEQ ID NO: 50 - protein, 14 aa, Homo sapiens
QTWDGNPTHGETNV

SEQ ID NO: 51 - DNA, 351 bp, Homo sapiens
gaggtgcagctgctggagagcggcggagggctggtgcagccaggcggcagcctgaggctgtcctgcgccgcctccggattcaccttcagcagctacgccatgaactgggtgcggcaggccccaggcaagggcctggagtgggtgtccaccatcagctacagcgggtcgctgatcagctacgccgacagcgtgaagggcaggttcaccatcagcagggacaacagcaagaacaccctgtacctgcagatgaacagcctgagggccgaggacaccgccgtgtactactgcgcccgcatccaccacgaccctatggatgtgtggggccagggcaccctggtgacagtgagctca

SEQ ID NO: 52 - protein, 117 aa, Homo sapiens
EVQLLESGGGLVQPGGSLRLSCAASGFTFSSYAMNWVRQAPGKGLEWVSTISYSGSLISYADSVKGRFTISRDNSKNTLYLQMNSLRAEDTAVYYCARIHHDPMDVWGQGTLVTVSS

SEQ ID NO: 53 - protein, 5 aa, Homo sapiens
SYAMN

SEQ ID NO: 54 - protein, 17 aa, Homo sapiens
TISYSGSLISYADSVKG

SEQ ID NO: 55 - protein, 8 aa, Homo sapiens
IHHDPMDV

SEQ ID NO: 56 - DNA, 333 bp, Homo sapiens; identical to SEQ ID NO: 16

SEQ ID NO: 57 - protein, 111 aa, Homo sapiens; identical to SEQ ID NO: 7

SEQ ID NO: 58 - protein, 11 aa, Homo sapiens
SGDNLGKKYVQ

SEQ ID NO: 59 - protein, 7 aa, Homo sapiens
DDSNRPS

SEQ ID NO: 60 - protein, 14 aa, Homo sapiens
QTWDGNPTTGETNV

SEQ ID NO: 61 - DNA, 351 bp, Homo sapiens
gaggtgcagctgctggagagcggcggagggctggtgcagccaggcggcagcctgaggctgtcctgcgccgcctccggattcaccttcagcagctacgccatgaactgggtgcggcaggccccaggcaagggcctggagtgggtgtccaccatcagctacagcgggtcgctgatcagctacgccgacagcgtgaagggcaggttcaccatcagcagggacaacagcaagaacaccctgtacctgcagatgaacagcctgagggccgaggacaccgccgtgtactactgcgcccgcatccaccacgaccctatggatcactggggccagggcaccctggtgacagtgagctca

SEQ ID NO: 62 - protein, 117 aa, Homo sapiens
EVQLLESGGGLVQPGGSLRLSCAASGFTFSSYAMNWVRQAPGKGLEWVSTISYSGSLISYADSVKGRFTISRDNSKNTLYLQMNSLRAEDTAVYYCARIHHDPMDHWGQGTLVTVSS

SEQ ID NO: 63 - protein, 5 aa, Homo sapiens
SYAMN

SEQ ID NO: 64 - protein, 17 aa, Homo sapiens
TISYSGSLISYADSVKG

SEQ ID NO: 65 - protein, 8 aa, Homo sapiens
IHHDPMDH

SEQ ID NO: 66 - DNA, 333 bp, Homo sapiens; identical to SEQ ID NO: 16

SEQ ID NO: 67 - protein, 111 aa, Homo sapiens; identical to SEQ ID NO: 7

SEQ ID NO: 68 - protein, 11 aa, Homo sapiens
SGDNLGKKYVQ

SEQ ID NO: 69 - protein, 7 aa, Homo sapiens
DDSNRPS

SEQ ID NO: 70 - protein, 14 aa, Homo sapiens
QTWDGNPTTGETNV

SEQ ID NO: 71 - DNA, 351 bp, Homo sapiens
gaggtgcagctgctggagagcggcggagggctggtgcagccaggcggcagcctgaggctgtcctgcgccgcctccggattcaccttcagcagctacgccatgaactgggtgcggcaggccccaggcaagggcctggagtgggtgtccaccatcagctacagcgggtcgctgatcagctacgccgacagcgtgaagggcaggttcaccatcagcagggacaacagcaagaacaccctgtacctgcagatgaacagcctgagggccgaggacaccgccgtgtactactgcgcccgcatcaacaacgaccctatggatgtgtggggccagggcaccctggtgacagtgagctca

SEQ ID NO: 72 - protein, 117 aa, Homo sapiens; identical to SEQ ID NO: 2

SEQ ID NO: 73 - protein, 5 aa, Homo sapiens
SYAMN

SEQ ID NO: 74 - protein, 17 aa, Homo sapiens
TISYSGSLISYADSVKG

SEQ ID NO: 75 - protein, 8 aa, Homo sapiens
INNDPMDV

SEQ ID NO: 76 - DNA, 333 bp, Homo sapiens
agtatcgagctgacccagccccccagcgtgagcgtgtccccaggccagaccgccagcatcacctgcagcggcgacaacctgggcaagaaatacgtgcagtggtatcagcagaagcccggccagtcccccgtgctggtgatctacgacgacagcaacaggcccagcggcatccccgagaggttcagcggcagcaacagcggcaacaccgccaccctgaccatcagcggcacccaggcgatggacgaggccgactactactgccacacctggcaccacaacccgcacacgggggagaccaaccacttcggcggagggaccaagttaaccgtccta

SEQ ID NO: 77 - protein, 111 aa, Homo sapiens
SIELTQPPSVSVSPGQTASITCSGDNLGKKYVQWYQQKPGQSPVLVIYDDSNRPSGIPERFSGSNSGNTATLTISGTQAMDEADYYCHTWHHNPHTGETNHFGGGTKLTVL

SEQ ID NO: 78 - protein, 11 aa, Homo sapiens
SGDNLGKKYVQ

SEQ ID NO: 79 - protein, 7 aa, Homo sapiens
DDSNRPS

SEQ ID NO: 80 - protein, 14 aa, Homo sapiens
HTWHHNPHTGETNH

SEQ ID NO: 81 - DNA, 351 bp, Homo sapiens; identical to SEQ ID NO: 71

SEQ ID NO: 82 - protein, 117 aa, Homo sapiens; identical to SEQ ID NO: 2

SEQ ID NO: 83 - protein, 5 aa, Homo sapiens
SYAMN

SEQ ID NO: 84 - protein, 17 aa, Homo sapiens
TISYSGSLISYADSVKG

SEQ ID NO: 85 - protein, 8 aa, Homo sapiens
INNDPMDV

SEQ ID NO: 86 - DNA, 333 bp, Homo sapiens
agtatcgagctgacccagccccccagcgtgagcgtgtccccaggccagaccgccagcatcacctgcagcggcgacaacctgggcaagaaatacgtgcagtggtatcagcagaagcccggccagtcccccgtgctggtgatctacgacgacagcaacaggcccagcggcatccccgagaggttcagcggcagcaacagcggcaacaccgccaccctgaccatcagcggcacccaggcgatggacgaggccgactactactgccaccactggcacgggaaccaccacacgggggagaccaaccacttcggcggagggaccaagttaaccgtccta

SEQ ID NO: 87 - protein, 111 aa, Homo sapiens
SIELTQPPSVSVSPGQTASITCSGDNLGKKYVQWYQQKPGQSPVLVIYDDSNRPSGIPERFSGSNSGNTATLTISGTQAMDEADYYCHHWHGNHHTGETNHFGGGTKLTVL

SEQ ID NO: 88 - protein, 11 aa, Homo sapiens
SGDNLGKKYVQ

SEQ ID NO: 89 - protein, 7 aa, Homo sapiens
DDSNRPS

SEQ ID NO: 90 - protein, 14 aa, Homo sapiens
HHWHGNHHTGETNH

SEQ ID NO: 91 - DNA, 351 bp, Homo sapiens; identical to SEQ ID NO: 71

SEQ ID NO: 92 - protein, 117 aa, Homo sapiens; identical to SEQ ID NO: 2

SEQ ID NO: 93 - protein, 5 aa, Homo sapiens
SYAMN

SEQ ID NO: 94 - protein, 17 aa, Homo sapiens
TISYSGSLISYADSVKG

SEQ ID NO: 95 - protein, 8 aa, Homo sapiens
INNDPMDV

SEQ ID NO: 96 - DNA, 333 bp, Homo sapiens
agtatcgagctgacccagccccccagcgtgagcgtgtccccaggccagaccgccagcatcacctgcagcggcgacaacctgggcaagaaatacgtgcagtggtatcagcagaagcccggccagtcccccgtgctggtgatctacgacgacagcaacaggcccagcggcatccccgagaggttcagcggcagcaacagcggcaacaccgccaccctgaccatcagcggcacccaggcgatggacgaggccgactactactgccacacctggcaccaccacccgacgcatggggagcacaacgtgttcggcggagggaccaagttaaccgtccta

SEQ ID NO: 97 - protein, 111 aa, Homo sapiens
SIELTQPPSVSVSPGQTASITCSGDNLGKKYVQWYQQKPGQSPVLVIYDDSNRPSGIPERFSGSNSGNTATLTISGTQAMDEADYYCHTWHHHPTHGEHNVFGGGTKLTVL

SEQ ID NO: 98 - protein, 11 aa, Homo sapiens
SGDNLGKKYVQ

SEQ ID NO: 99 - protein, 7 aa, Homo sapiens
DDSNRPS

SEQ ID NO: 100 - protein, 14 aa, Homo sapiens
HTWHHHPTHGEHNV

SEQ ID NO: 101 - DNA, 351 bp, Homo sapiens; identical to SEQ ID NO: 71

SEQ ID NO: 102 - protein, 117 aa, Homo sapiens; identical to SEQ ID NO: 2

SEQ ID NO: 103 - protein, 5 aa, Homo sapiens
SYAMN

SEQ ID NO: 104 - protein, 17 aa, Homo sapiens
TISYSGSLISYADSVKG

SEQ ID NO: 105 - protein, 8 aa, Homo sapiens
INNDPMDV

SEQ ID NO: 106 - DNA, 333 bp, Homo sapiens
agtatcgagctgacccagccccccagcgtgagcgtgtccccaggccagaccgccagcatcacctgcagcggcgacaacctgggcaagaaatacgtgcagtggtatcagcagaagcccggccagtcccccgtgctggtgatctacgacgacagcaacaggcccagcggcatccccgagaggttcagcggcagcaacagcggcaacaccgccaccctgaccatcagcggcacccaggcgatggacgaggccgactactactgccagacctgggacgggcaccacacgcatggggagcaccacgtgttcggcggagggaccaagttaaccgtccta

SEQ ID NO: 107 - protein, 111 aa, Homo sapiens
SIELTQPPSVSVSPGQTASITCSGDNLGKKYVQWYQQKPGQSPVLVIYDDSNRPSGIPERFSGSNSGNTATLTISGTQAMDEADYYCQTWDGHHTHGEHHVFGGGTKLTVL

SEQ ID NO: 108 - protein, 11 aa, Homo sapiens
SGDNLGKKYVQ

SEQ ID NO: 109 - protein, 7 aa, Homo sapiens
DDSNRPS

SEQ ID NO: 110 - protein, 14 aa, Homo sapiens
QTWDGHHTHGEHHV

SEQ ID NO: 111 - DNA, 351 bp, Homo sapiens; identical to SEQ ID NO: 71

SEQ ID NO: 112 - protein, 117 aa, Homo sapiens; identical to SEQ ID NO: 2

SEQ ID NO: 113 - protein, 5 aa, Homo sapiens
SYAMN

SEQ ID NO: 114 - protein, 17 aa, Homo sapiens
TISYSGSLISYADSVKG

SEQ ID NO: 115 - protein, 8 aa, Homo sapiens
INNDPMDV

SEQ ID NO: 116 - DNA, 333 bp, Homo sapiens
agtatcgagctgacccagccccccagcgtgagcgtgtccccaggccagaccgccagcatcacctgcagcggcgacaacctgggcaagaaatacgtgcagtggtatcagcagaagcccggccagtcccccgtgctggtgatctacgacgacagcaacaggcccagcggcatccccgagaggttcagcggcagcaacagcggcaacaccgccaccctgaccatcagcggcacccaggcgatggacgaggccgactactactgccagacctgggaccacaaccaccacacggggcacaccaacgtgttcggcggagggaccaagttaaccgtccta

SEQ ID NO: 117 - protein, 111 aa, Homo sapiens
SIELTQPPSVSVSPGQTASITCSGDNLGKKYVQWYQQKPGQSPVLVIYDDSNRPSGIPERFSGSNSGNTATLTISGTQAMDEADYYCQTWDHNHHTGHTNVFGGGTKLTVL

SEQ ID NO: 118 - protein, 11 aa, Homo sapiens
SGDNLGKKYVQ

SEQ ID NO: 119 - protein, 7 aa, Homo sapiens
DDSNRPS

SEQ ID NO: 120 - protein, 14 aa, Homo sapiens
QTWDHNHHTGHTNV

SEQ ID NO: 121 - DNA, 351 bp, Homo sapiens; identical to SEQ ID NO: 71

SEQ ID NO: 122 - protein, 117 aa, Homo sapiens; identical to SEQ ID NO: 2

SEQ ID NO: 123 - protein, 5 aa, Homo sapiens
SYAMN

SEQ ID NO: 124 - protein, 17 aa, Homo sapiens
TISYSGSLISYADSVKG

SEQ ID NO: 125 - protein, 8 aa, Homo sapiens
INNDPMDV

SEQ ID NO: 126 - DNA, 333 bp, Homo sapiens
agtatcgagctgacccagccccccagcgtgagcgtgtccccaggccagaccgccagcatcacctgcagcggcgacaacctgggcaagaaatacgtgcagtggtatcagcagaagcccggccagtcccccgtgctggtgatctacgacgacagcaacaggcccagcggcatccccgagaggttcagcggcagcaacagcggcaacaccgccaccctgaccatcagcggcacccaggcgatggacgaggccgactactactgccacacctggcaccaccaccaccacacgggggagcacaaccacttcggcggagggaccaagttaaccgtccta

SEQ ID NO: 127 - protein, 111 aa, Homo sapiens
SIELTQPPSVSVSPGQTASITCSGDNLGKKYVQWYQQKPGQSPVLVIYDDSNRPSGIPERFSGSNSGNTATLTISGTQAMDEADYYCHTWHHHHHTGEHNHFGGGTKLTVL

SEQ ID NO: 128 - protein, 11 aa, Homo sapiens
SGDNLGKKYVQ

SEQ ID NO: 129 - protein, 7 aa, Homo sapiens
DDSNRPS

SEQ ID NO: 130 - protein, 14 aa, Homo sapiens
HTWHHHHHTGEHNH

SEQ ID NO: 131 - DNA, 351 bp, Homo sapiens; identical to SEQ ID NO: 71

SEQ ID NO: 132 - protein, 117 aa, Homo sapiens; identical to SEQ ID NO: 2

SEQ ID NO: 133 - protein, 5 aa, Homo sapiens
SYAMN

SEQ ID NO: 134 - protein, 17 aa, Homo sapiens
TISYSGSLISYADSVKG

SEQ ID NO: 135 - protein, 8 aa, Homo sapiens
INNDPMDV

SEQ ID NO: 136 - DNA, 333 bp, Homo sapiens
agtatcgagctgacccagccccccagcgtgagcgtgtccccaggccagaccgccagcatcacctgcagcggcgacaacctgggcaagaaatacgtgcagtggtatcagcagaagcccggccagtcccccgtgctggtgatctacgacgacagcaacaggcccagcggcatccccgagaggttcagcggcagcaacagcggcaacaccgccaccctgaccatcagcggcacccaggcgatggacgaggccgactactactgccagcactggcacgggcacccgcaccatggggagcacaacgtgttcggcggagggaccaagttaaccgtccta

SEQ ID NO: 137 - protein, 111 aa, Homo sapiens
SIELTQPPSVSVSPGQTASITCSGDNLGKKYVQWYQQKPGQSPVLVIYDDSNRPSGIPERFSGSNSGNTATLTISGTQAMDEADYYCQHWHGHPHHGEHNVFGGGTKLTVL

SEQ ID NO: 138 - protein, 11 aa, Homo sapiens
SGDNLGKKYVQ

SEQ ID NO: 139 - protein, 7 aa, Homo sapiens
DDSNRPS

SEQ ID NO: 140 - protein, 14 aa, Homo sapiens
QHWHGHPHHGEHNV

SEQ ID NO: 141 - DNA, 351 bp, Homo sapiens; identical to SEQ ID NO: 71

SEQ ID NO: 142 - protein, 117 aa, Homo sapiens; identical to SEQ ID NO: 2

SEQ ID NO: 143 - protein, 5 aa, Homo sapiens
SYAMN

SEQ ID NO: 144 - protein, 17 aa, Homo sapiens
TISYSGSLISYADSVKG

SEQ ID NO: 145 - protein, 8 aa, Homo sapiens
INNDPMDV

SEQ ID NO: 146 - DNA, 333 bp, Homo sapiens
agtatcgagctgacccagccccccagcgtgagcgtgtccccaggccagaccgccagcatcacctgcagcggcgacaacctgggcaagaaatacgtgcagtggtatcagcagaagcccggccagtcccccgtgctggtgatctacgacgacagcaacaggcccagcggcatccccgagaggttcagcggcagcaacagcggcaacaccgccaccctgaccatcagcggcacccaggcgatggacgaggccgactactactgccagcactgggacgggaaccaccaccatggggagaccaaccacttcggcggagggaccaagttaaccgtccta

SEQ ID NO: 147 - protein, 111 aa, Homo sapiens
SIELTQPPSVSVSPGQTASITCSGDNLGKKYVQWYQQKPGQSPVLVIYDDSNRPSGIPERFSGSNSGNTATLTISGTQAMDEADYYCQHWDGNHHHGETNHFGGGTKLTVL

SEQ ID NO: 148 - protein, 11 aa, Homo sapiens
SGDNLGKKYVQ

SEQ ID NO: 149 - protein, 7 aa, Homo sapiens
DDSNRPS

SEQ ID NO: 150 - protein, 14 aa, Homo sapiens
QHWDGNHHHGETNH

SEQ ID NO: 151 - DNA, 351 bp, Homo sapiens; identical to SEQ ID NO: 71

SEQ ID NO: 152 - protein, 117 aa, Homo sapiens; identical to SEQ ID NO: 2

SEQ ID NO: 153 - protein, 5 aa, Homo sapiens
SYAMN

SEQ ID NO: 154 - protein, 17 aa, Homo sapiens
TISYSGSLISYADSVKG

SEQ ID NO: 155 - protein, 8 aa, Homo sapiens
INNDPMDV

SEQ ID NO: 156 - DNA, 333 bp, Homo sapiens
agtatcgagctgacccagccccccagcgtgagcgtgtccccaggccagaccgccagcatcacctgcagcggcgacaacctgggcaagaaatacgtgcagtggtatcagcagaagcccggccagtcccccgtgctggtgatctacgacgacagcaacaggcccagcggcatccccgagaggttcagcggcagcaacagcggcaacaccgccaccctgaccatcagcggcacccaggcgatggacgaggccgactactactgccacacctgggaccaccaccacacgacgggggagcacaacgtgttcggcggagggaccaagttaaccgtccta

SEQ ID NO: 157 - protein, 111 aa, Homo sapiens
SIELTQPPSVSVSPGQTASITCSGDNLGKKYVQWYQQKPGQSPVLVIYDDSNRPSGIPERFSGSNSGNTATLTISGTQAMDEADYYCHTWDHHHTTGEHNVFGGGTKLTVL

SEQ ID NO: 158 - protein, 11 aa, Homo sapiens
SGDNLGKKYVQ

SEQ ID NO: 159 - protein, 7 aa, Homo sapiens
DDSNRPS

SEQ ID NO: 160 - protein, 14 aa, Homo sapiens
HTWDHHHTTGEHNV

SEQ ID NO: 161 - DNA, 351 bp, Homo sapiens; identical to SEQ ID NO: 71

SEQ ID NO: 162 - protein, 117 aa, Homo sapiens; identical to SEQ ID NO: 2

SEQ ID NO: 163 - protein, 5 aa, Homo sapiens
SYAMN

SEQ ID NO: 164 - protein, 17 aa, Homo sapiens
TISYSGSLISYADSVKG

SEQ ID NO: 165 - protein, 8 aa, Homo sapiens
INNDPMDV

SEQ ID NO: 166 - DNA, 333 bp, Homo sapiens
agtatcgagctgacccagccccccagcgtgagcgtgtccccaggccagaccgccagcatcacctgcagcggcgacaacctgggcaagaaatacgtgcagtggtatcagcagaagcccggccagtcccccgtgctggtgatctacgacgacagcaacaggcccagcggcatccccgagaggttcagcggcagcaacagcggcaacaccgccaccctgaccatcagcggcacccaggcgatggacgaggccgactactactgccaccactggcacgggcaccacacgacgggggagaccaaccacttcggcggagggaccaagttaaccgtccta

SEQ ID NO: 167 - protein, 111 aa, Homo sapiens
SIELTQPPSVSVSPGQTASITCSGDNLGKKYVQWYQQKPGQSPVLVIYDDSNRPSGIPERFSGSNSGNTATLTISGTQAMDEADYYCHHWHGHHTTGETNHFGGGTKLTVL

SEQ ID NO: 168 - protein, 11 aa, Homo sapiens
SGDNLGKKYVQ

SEQ ID NO: 169 - protein, 7 aa, Homo sapiens
DDSNRPS

SEQ ID NO: 170 - protein, 14 aa, Homo sapiens
HHWHGHHTTGETNH

SEQ ID NO: 171 - DNA, 351 bp, Homo sapiens; identical to SEQ ID NO: 71

SEQ ID NO: 172 - protein, 117 aa, Homo sapiens; identical to SEQ ID NO: 2

SEQ ID NO: 173 - protein, 5 aa, Homo sapiens
SYAMN

SEQ ID NO: 174 - protein, 17 aa, Homo sapiens
TISYSGSLISYADSVKG

SEQ ID NO: 175 - protein, 8 aa, Homo sapiens
INNDPMDV

SEQ ID NO: 176 - DNA, 333 bp, Homo sapiens
agtatcgagctgacccagccccccagcgtgagcgtgtccccaggccagaccgccagcatcacctgcagcggcgacaacctgggcaagaaatacgtgcagtggtatcagcagaagcccggccagtcccccgtgctggtgatctacgacgacagcaacaggcccagcggcatccccgagaggttcagcggcagcaacagcggcaacaccgccaccctgaccatcagcggcacccaggcgatggacgaggccgactactactgccaccactggcacgggcacccgcacacgggggagcacaacgtgttcggcggagggaccaagttaaccgtccta

SEQ ID NO: 177 - protein, 111 aa, Homo sapiens
SIELTQPPSVSVSPGQTASITCSGDNLGKKYVQWYQQKPGQSPVLVIYDDSNRPSGIPERFSGSNSGNTATLTISGTQAMDEADYYCHHWHGHPHTGEHNVFGGGTKLTVL

SEQ ID NO: 178 - protein, 11 aa, Homo sapiens
SGDNLGKKYVQ

SEQ ID NO: 179 - protein, 7 aa, Homo sapiens
DDSNRPS

SEQ ID NO: 180 - protein, 14 aa, Homo sapiens
HHWHGHPHTGEHNV

SEQ ID NO: 181 - DNA, 351 bp, Homo sapiens; identical to SEQ ID NO: 71

SEQ ID NO: 182 - protein, 117 aa, Homo sapiens; identical to SEQ ID NO: 2

SEQ ID NO: 183 - protein, 5 aa, Homo sapiens
SYAMN

SEQ ID NO: 184 - protein, 17 aa, Homo sapiens
TISYSGSLISYADSVKG

SEQ ID NO: 185 - protein, 8 aa, Homo sapiens
INNDPMDV

SEQ ID NO: 186 - DNA, 333 bp, Homo sapiens
agtatcgagctgacccagccccccagcgtgagcgtgtccccaggccagaccgccagcatcacctgcagcggcgacaacctgggcaagaaatacgtgcagtggtatcagcagaagcccggccagtcccccgtgctggtgatctacgacgacagcaacaggcccagcggcatccccgagaggttcagcggcagcaacagcggcaacaccgccaccctgaccatcagcggcacccaggcgatggacgaggccgactactactgccagcactgggacgggcaccacacgacgggggagaccaaccacttcggcggagggaccaagttaaccgtccta

SEQ ID NO: 187 - protein, 111 aa, Homo sapiens
SIELTQPPSVSVSPGQTASITCSGDNLGKKYVQWYQQKPGQSPVLVIYDDSNRPSGIPERFSGSNSGNTATLTISGTQAMDEADYYCQHWDGHHTTGETNHFGGGTKLTVL

SEQ ID NO: 188 - protein, 11 aa, Homo sapiens
SGDNLGKKYVQ

SEQ ID NO: 189 - protein, 7 aa, Homo sapiens
DDSNRPS

SEQ ID NO: 190 - protein, 14 aa, Homo sapiens
QHWDGHHTTGETNH

SEQ ID NO: 191 - DNA, 351 bp, Homo sapiens; identical to SEQ ID NO: 71

SEQ ID NO: 192 - protein, 117 aa, Homo sapiens; identical to SEQ ID NO: 2

SEQ ID NO: 193 - protein, 5 aa, Homo sapiens
SYAMN

SEQ ID NO: 194 - protein, 17 aa, Homo sapiens
TISYSGSLISYADSVKG

SEQ ID NO: 195 - protein, 8 aa, Homo sapiens
INNDPMDV

SEQ ID NO: 196 - DNA, 333 bp, Homo sapiens
agtatcgagctgacccagccccccagcgtgagcgtgtccccaggccagaccgccagcatcacctgcagcggcgacaacctgggcaagaaatacgtgcagtggtatcagcagaagcccggccagtcccccgtgctggtgatctacgacgacagcaacaggcccagcggcatccccgagaggttcagcggcagcaacagcggcaacaccgccaccctgaccatcagcggcacccaggcgatggacgaggccgactactactgccagacctgggacgggcaccaccacacgggggagaccaaccacttcggcggagggaccaagttaaccgtccta

SEQ ID NO: 197 - protein, 111 aa, Homo sapiens
SIELTQPPSVSVSPGQTASITCSGDNLGKKYVQWYQQKPGQSPVLVIYDDSNRPSGIPERFSGSNSGNTATLTISGTQAMDEADYYCQTWDGHHHTGETNHFGGGTKLTVL

SEQ ID NO: 198 - protein, 11 aa, Homo sapiens
SGDNLGKKYVQ

SEQ ID NO: 199 - protein, 7 aa, Homo sapiens
DDSNRPS

SEQ ID NO: 200 - protein, 14 aa, Homo sapiens
QTWDGHHHTGETNH

SEQ ID NO: 201 - DNA, 351 bp, Homo sapiens
gaggtgcagctgctggagagcggcggagggctggtgcagccaggcggcagcctgaggctgtcctgcgccgcctccggattcaccttcagcagctacgccatgaactgggtgcggcaggccccaggcaagggcctggagtgggtgtccaccatcagccacagcgggcaccacatcagccaccacgacagccatcatggcaggttcaccatcagcagggacaacagcaagaacaccctgtacctgcagatgaacagcctgagggccgaggacaccgccgtgtactactgcgcccgcatcaacaacgaccctatggatgtgtggggccagggcaccctggtgacagtgagctca

SEQ ID NO: 202 - protein, 117 aa, Homo sapiens
EVQLLESGGGLVQPGGSLRLSCAASGFTFSSYAMNWVRQAPGKGLEWVSTISHSGHHISHHDSHHGRFTISRDNSKNTLYLQMNSLRAEDTAVYYCARINNDPMDVWGQGTLVTVSS

SEQ ID NO: 203 - protein, 5 aa, Homo sapiens
SYAMN

SEQ ID NO: 204 - protein, 17 aa, Homo sapiens
TISHSGHHISHHDSHHG

SEQ ID NO: 205 - protein, 8 aa, Homo sapiens
INNDPMDV

SEQ ID NO: 206 - DNA, 333 bp, Homo sapiens; identical to SEQ ID NO: 16

SEQ ID NO: 207 - protein, 111 aa, Homo sapiens; identical to SEQ ID NO: 7

SEQ ID NO: 208 - protein, 11 aa, Homo sapiens
SGDNLGKKYVQ

SEQ ID NO: 209 - protein, 7 aa, Homo sapiens
DDSNRPS

SEQ ID NO: 210 - protein, 14 aa, Homo sapiens
QTWDGNPTTGETNV

SEQ ID NO: 211 - DNA, 351 bp, Homo sapiens
gaggtgcagctgctggagagcggcggagggctggtgcagccaggcggcagcctgaggctgtcctgcgccgcctccggattcaccttcagcagctacgccatgaactgggtgcggcaggccccaggcaagggcctggagtgggtgtccaccatcagccacagccactcgctgatcagctacgcccacagcgtgcatggcaggttcaccatcagcagggacaacagcaagaacaccctgtacctgcagatgaacagcctgagggccgaggacaccgccgtgtactactgcgcccgcatcaacaacgaccctatggatgtgtggggccagggcaccctggtgacagtgagctca

SEQ ID NO: 212 - protein, 117 aa, Homo sapiens
EVQLLESGGGLVQPGGSLRLSCAASGFTFSSYAMNWVRQAPGKGLEWVSTISHSHSLISYAHSVHGRFTISRDNSKNTLYLQMNSLRAEDTAVYYCARINNDPMDVWGQGTLVTVSS

SEQ ID NO: 213 - protein, 5 aa, Homo sapiens
SYAMN

SEQ ID NO: 214 - protein, 17 aa, Homo sapiens
TISHSHSLISYAHSVHG

SEQ ID NO: 215 - protein, 8 aa, Homo sapiens
INNDPMDV

SEQ ID NO: 216 - DNA, 333 bp, Homo sapiens; identical to SEQ ID NO: 16

SEQ ID NO: 217 - protein, 111 aa, Homo sapiens; identical to SEQ ID NO: 7

SEQ ID NO: 218 - protein, 11 aa, Homo sapiens
SGDNLGKKYVQ

SEQ ID NO: 219 - protein, 7 aa, Homo sapiens
DDSNRPS

SEQ ID NO: 220 - protein, 14 aa, Homo sapiens
QTWDGNPTTGETNV

SEQ ID NO: 221 - DNA, 351 bp, Homo sapiens
gaggtgcagctgctggagagcggcggagggctggtgcagccaggcggcagcctgaggctgtcctgcgccgcctccggattcaccttcagcagctacgccatgaactgggtgcggcaggccccaggcaagggcctggagtgggtgtccaccatccaccacagcgggcacctgcacagccacgccgaccacgtgaagggcaggttcaccatcagcagggacaacagcaagaacaccctgtacctgcagatgaacagcctgagggccgaggacaccgccgtgtactactgcgcccgcatcaacaacgaccctatggatgtgtggggccagggcaccctggtgacagtgagctca

SEQ ID NO: 222 - protein, 117 aa, Homo sapiens
EVQLLESGGGLVQPGGSLRLSCAASGFTFSSYAMNWVRQAPGKGLEWVSTIHHSGHLHSHADHVKGRFTISRDNSKNTLYLQMNSLRAEDTAVYYCARINNDPMDVWGQGTLVTVSS

SEQ ID NO: 223 - protein, 5 aa, Homo sapiens
SYAMN

SEQ ID NO: 224 - protein, 17 aa, Homo sapiens
TIHHSGHLHSHADHVKG

SEQ ID NO: 225 - protein, 8 aa, Homo sapiens
INNDPMDV

SEQ ID NO: 226 - DNA, 333 bp, Homo sapiens; identical to SEQ ID NO: 16

SEQ ID NO: 227 - protein, 111 aa, Homo sapiens; identical to SEQ ID NO: 7

SEQ ID NO: 228 - protein, 11 aa, Homo sapiens
SGDNLGKKYVQ

SEQ ID NO: 229 - protein, 7 aa, Homo sapiens
DDSNRPS

SEQ ID NO: 230 - protein, 14 aa, Homo sapiens
QTWDGNPTTGETNV

SEQ ID NO: 231 - DNA, 351 bp, Homo sapiens
gaggtgcagctgctggagagcggcggagggctggtgcagccaggcggcagcctgaggctgtcctgcgccgcctccggattcaccttcagcagctacgccatgaactgggtgcggcaggccccaggcaagggcctggagtgggtgtccaccatcagccacagcgggcacctgatccaccacgccgacagccataagggcaggttcaccatcagcagggacaacagcaagaacaccctgtacctgcagatgaacagcctgagggccgaggacaccgccgtgtactactgcgcccgcatcaacaacgaccctatggatgtgtggggccagggcaccctggtgacagtgagctca

SEQ ID NO: 232 - protein, 117 aa, Homo sapiens
EVQLLESGGGLVQPGGSLRLSCAASGFTFSSYAMNWVRQAPGKGLEWVSTISHSGHLIHHADSHKGRFTISRDNSKNTLYLQMNSLRAEDTAVYYCARINNDPMDVWGQGTLVTVSS

SEQ ID NO: 233 - protein, 5 aa, Homo sapiens
SYAMN

SEQ ID NO: 234 - protein, 17 aa, Homo sapiens
TISHSGHLIHHADSHKG

SEQ ID NO: 235 - protein, 8 aa, Homo sapiens
INNDPMDV

SEQ ID NO: 236 - DNA, 333 bp, Homo sapiens; identical to SEQ ID NO: 16

SEQ ID NO: 237 - protein, 111 aa, Homo sapiens; identical to SEQ ID NO: 7

SEQ ID NO: 238 - protein, 11 aa, Homo sapiens
SGDNLGKKYVQ

SEQ ID NO: 239 - protein, 7 aa, Homo sapiens
DDSNRPS

SEQ ID NO: 240 - protein, 14 aa, Homo sapiens
QTWDGNPTTGETNV

SEQ ID NO: 241 - DNA, 351 bp, Homo sapiens
gaggtgcagctgctggagagcggcggagggctggtgcagccaggcggcagcctgaggctgtcctgcgccgcctccggattcaccttcagcagctacgccatgaactgggtgcggcaggccccaggcaagggcctggagtgggtgtccaccatcagctaccacgggtcgcacatcagctaccaccacagccataagggcaggttcaccatcagcagggacaacagcaagaacaccctgtacctgcagatgaacagcctgagggccgaggacaccgccgtgtactactgcgcccgcatcaacaacgaccctatggatgtgtggggccagggcaccctggtgacagtgagctca

SEQ ID NO: 242 - protein, 117 aa, Homo sapiens
EVQLLESGGGLVQPGGSLRLSCAASGFTFSSYAMNWVRQAPGKGLEWVSTISYHGSHISYHHSHKGRFTISRDNSKNTLYLQMNSLRAEDTAVYYCARINNDPMDVWGQGTLVTVSS

SEQ ID NO: 243 - protein, 5 aa, Homo sapiens
SYAMN

SEQ ID NO: 244 - protein, 17 aa, Homo sapiens
TISYHGSHISYHHSHKG

SEQ ID NO: 245 - protein, 8 aa, Homo sapiens
INNDPMDV

SEQ ID NO: 246 - DNA, 333 bp, Homo sapiens; identical to SEQ ID NO: 16

SEQ ID NO: 247 - protein, 111 aa, Homo sapiens; identical to SEQ ID NO: 7

SEQ ID NO: 248 - protein, 11 aa, Homo sapiens
SGDNLGKKYVQ

SEQ ID NO: 249 - protein, 7 aa, Homo sapiens
DDSNRPS

SEQ ID NO: 250 - protein, 14 aa, Homo sapiens
QTWDGNPTTGETNV

SEQ ID NO: 251 - DNA, 351 bp, Homo sapiens
gaggtgcagctgctggagagcggcggagggctggtgcagccaggcggcagcctgaggctgtcctgcgccgcctccggattcaccttcagcagctacgccatgaactgggtgcggcaggccccaggcaagggcctggagtgggtgtccaccatcagctaccacgggtcgcacatcagctacgccgaccaccataagcacaggttcaccatcagcagggacaacagcaagaacaccctgtacctgcagatgaacagcctgagggccgaggacaccgccgtgtactactgcgcccgcatcaacaacgaccctatggatgtgtggggccagggcaccctggtgacagtgagctca

SEQ ID NO: 252 - protein, 117 aa, Homo sapiens
EVQLLESGGGLVQPGGSLRLSCAASGFTFSSYAMNWVRQAPGKGLEWVSTISYHGSHISYADHHKHRFTISRDNSKNTLYLQMNSLRAEDTAVYYCARINNDPMDVWGQGTLVTVSS

SEQ ID NO: 253 - protein, 5 aa, Homo sapiens
SYAMN

SEQ ID NO: 254 - protein, 17 aa, Homo sapiens
TISYHGSHISYADHHKH

SEQ ID NO: 255 - protein, 8 aa, Homo sapiens
INNDPMDV

SEQ ID NO: 256 - DNA, 333 bp, Homo sapiens; identical to SEQ ID NO: 16

SEQ ID NO: 257 - protein, 111 aa, Homo sapiens; identical to SEQ ID NO: 7

SEQ ID NO: 258 - protein, 11 aa, Homo sapiens
SGDNLGKKYVQ

SEQ ID NO: 259 - protein, 7 aa, Homo sapiens
DDSNRPS

SEQ ID NO: 260 - protein, 14 aa, Homo sapiens
QTWDGNPTTGETNV

SEQ ID NO: 261 - DNA, 351 bp, Homo sapiens
gaggtgcagctgctggagagcggcggagggctggtgcagccaggcggcagcctgaggctgtcctgcgccgcctccggattcaccttcagcagctacgccatgaactgggtgcggcaggccccaggcaagggcctggagtgggtgtccaccatcagctacagcgggcacctgatccactacgccgaccaccatcatggcaggttcaccatcagcagggacaacagcaagaacaccctgtacctgcagatgaacagcctgagggccgaggacaccgccgtgtactactgcgcccgcatcaacaacgaccctatggatgtgtggggccagggcaccctggtgacagtgagctca

SEQ ID NO: 262 - protein, 117 aa, Homo sapiens
EVQLLESGGGLVQPGGSLRLSCAASGFTFSSYAMNWVRQAPGKGLEWVSTISYSGHLIHYADHHHGRFTISRDNSKNTLYLQMNSLRAEDTAVYYCARINNDPMDVWGQGTLVTVSS

SEQ ID NO: 263 - protein, 5 aa, Homo sapiens
SYAMN

SEQ ID NO: 264 - protein, 17 aa, Homo sapiens
TISYSGHLIHYADHHHG

SEQ ID NO: 265 - protein, 8 aa, Homo sapiens
INNDPMDV

SEQ ID NO: 266 - DNA, 333 bp, Homo sapiens; identical to SEQ ID NO: 16

SEQ ID NO: 267 - protein, 111 aa, Homo sapiens; identical to SEQ ID NO: 7

SEQ ID NO: 268 - protein, 11 aa, Homo sapiens
SGDNLGKKYVQ

SEQ ID NO: 269 - protein, 7 aa, Homo sapiens
DDSNRPS

SEQ ID NO: 270 - protein, 14 aa, Homo sapiens
QTWDGNPTTGETNV

SEQ ID NO: 271 - DNA, 351 bp, Homo sapiens
gaggtgcagctgctggagagcggcggagggctggtgcagccaggcggcagcctgaggctgtcctgcgccgcctccggattcaccttcagcagctacgccatgaactgggtgcggcaggccccaggcaagggcctggagtgggtgtccaccatcagctaccacgggtcgcacatcagccacgccgaccacgtgcatggcaggttcaccatcagcagggacaacagcaagaacaccctgtacctgcagatgaacagcctgagggccgaggacaccgccgtgtactactgcgcccgcatcaacaacgaccctatggatgtgtggggccagggcaccctggtgacagtgagctca

SEQ ID NO: 272 - protein, 117 aa, Homo sapiens
EVQLLESGGGLVQPGGSLRLSCAASGFTFSSYAMNWVRQAPGKGLEWVSTISYHGSHISHADHVHGRFTISRDNSKNTLYLQMNSLRAEDTAVYYCARINNDPMDVWGQGTLVTVSS

SEQ ID NO: 273 - protein, 5 aa, Homo sapiens
SYAMN

SEQ ID NO: 274 - protein, 17 aa, Homo sapiens
TISYHGSHISHADHVHG

SEQ ID NO: 275 - protein, 8 aa, Homo sapiens
INNDPMDV

SEQ ID NO: 276 - DNA, 333 bp, Homo sapiens; identical to SEQ ID NO: 16

SEQ ID NO: 277 - protein, 111 aa, Homo sapiens; identical to SEQ ID NO: 7

SEQ ID NO: 278 - protein, 11 aa, Homo sapiens
SGDNLGKKYVQ

SEQ ID NO: 279 - protein, 7 aa, Homo sapiens
DDSNRPS

SEQ ID NO: 280 - protein, 14 aa, Homo sapiens
QTWDGNPTTGETNV

SEQ ID NO: 281 - DNA, 351 bp, Homo sapiens
gaggtgcagctgctggagagcggcggagggctggtgcagccaggcggcagcctgaggctgtcctgcgccgcctccggattcaccttcagcagctacgccatgaactgggtgcggcaggccccaggcaagggcctggagtgggtgtccaccatcagctaccacgggcaccacatcagccacgccgaccacgtgaagcacaggttcaccatcagcagggacaacagcaagaacaccctgtacctgcagatgaacagcctgagggccgaggacaccgccgtgtactactgcgcccgcatcaacaacgaccctatggatgtgtggggccagggcaccctggtgacagtgagctca

SEQ ID NO: 282 - protein, 117 aa, Homo sapiens
EVQLLESGGGLVQPGGSLRLSCAASGFTFSSYAMNWVRQAPGKGLEWVSTISYHGHHISHADHVKHRFTISRDNSKNTLYLQMNSLRAEDTAVYYCARINNDPMDVWGQGTLVTVSS

SEQ ID NO: 283 - protein, 5 aa, Homo sapiens
SYAMN

SEQ ID NO: 284 - protein, 17 aa, Homo sapiens
TISYHGHHISHADHVKH

SEQ ID NO: 285 - protein, 8 aa, Homo sapiens
INNDPMDV

SEQ ID NO: 286 - DNA, 333 bp, Homo sapiens; identical to SEQ ID NO: 16

SEQ ID NO: 287 - protein, 111 aa, Homo sapiens; identical to SEQ ID NO: 7

SEQ ID NO: 288 - protein, 11 aa, Homo sapiens
SGDNLGKKYVQ

SEQ ID NO: 289 - protein, 7 aa, Homo sapiens
DDSNRPS

SEQ ID NO: 290 - protein, 14 aa, Homo sapiens
QTWDGNPTTGETNV

SEQ ID NO: 291 - DNA, 351 bp, Homo sapiens
gaggtgcagctgctggagagcggcggagggctggtgcagccaggcggcagcctgaggctgtcctgcgccgcctccggattcaccttcagcagctacgccatgaactgggtgcggcaggccccaggcaagggcctggagtgggtgtccaccatcagccacagcgggcacctgatccaccaccaccacagcgtgaagggcaggttcaccatcagcagggacaacagcaagaacaccctgtacctgcagatgaacagcctgagggccgaggacaccgccgtgtactactgcgcccgcatcaacaacgaccctatggatgtgtggggccagggcaccctggtgacagtgagctca

SEQ ID NO: 292 - protein, 117 aa, Homo sapiens
EVQLLESGGGLVQPGGSLRLSCAASGFTFSSYAMNWVRQAPGKGLEWVSTISHSGHLIHHHHSVKGRFTISRDNSKNTLYLQMNSLRAEDTAVYYCARINNDPMDVWGQGTLVTVSS

SEQ ID NO: 293 - protein, 5 aa, Homo sapiens
SYAMN

SEQ ID NO: 294 - protein, 17 aa, Homo sapiens
TISHSGHLIHHHHSVKG

SEQ ID NO: 295 - protein, 8 aa, Homo sapiens
INNDPMDV

SEQ ID NO: 296 - DNA, 333 bp, Homo sapiens; identical to SEQ ID NO: 16

SEQ ID NO: 297 - protein, 111 aa, Homo sapiens; identical to SEQ ID NO: 7

SEQ ID NO: 298 - protein, 11 aa, Homo sapiens
SGDNLGKKYVQ

SEQ ID NO: 299 - protein, 7 aa, Homo sapiens
DDSNRPS

SEQ ID NO: 300 - protein, 14 aa, Homo sapiens
QTWDGNPTTGETNV

SEQ ID NO: 301 - DNA, 351 bp, Homo sapiens
gaggtgcagctgctggagagcggcggagggctggtgcagccaggcggcagcctgaggctgtcctgcgccgcctccggattcaccttcagcagctacgccatgaactgggtgcggcaggccccaggcaagggcctggagtgggtgtccaccatcagctaccacgggtcgcacatcagctaccacgacagccatcatggcaggttcaccatcagcagggacaacagcaagaacaccctgtacctgcagatgaacagcctgagggccgaggacaccgccgtgtactactgcgcccgcatcaacaacgaccctatggatgtgtggggccagggcaccctggtgacagtgagctca

SEQ ID NO: 302 - protein, 117 aa, Homo sapiens
EVQLLESGGGLVQPGGSLRLSCAASGFTFSSYAMNWVRQAPGKGLEWVSTISYHGSHISYHDSHHGRFTISRDNSKNTLYLQMNSLRAEDTAVYYCARINNDPMDVWGQGTLVTVSS

SEQ ID NO: 303 - protein, 5 aa, Homo sapiens
SYAMN

SEQ ID NO: 304 - protein, 17 aa, Homo sapiens
TISYHGSHISYHDSHHG

SEQ ID NO: 305 - protein, 8 aa, Homo sapiens
INNDPMDV

SEQ ID NO: 306 - DNA, 333 bp, Homo sapiens; identical to SEQ ID NO: 16

SEQ ID NO: 307 - protein, 111 aa, Homo sapiens; identical to SEQ ID NO: 7

SEQ ID NO: 308 - protein, 11 aa, Homo sapiens
SGDNLGKKYVQ

SEQ ID NO: 309 - protein, 7 aa, Homo sapiens
DDSNRPS

SEQ ID NO: 310 - protein, 14 aa, Homo sapiens
QTWDGNPTTGETNV

SEQ ID NO: 311 - DNA, 351 bp, Homo sapiens
gaggtgcagctgctggagagcggcggagggctggtgcagccaggcggcagcctgaggctgtcctgcgccgcctccggattcaccttcagcagctacgccatgaactgggtgcggcaggccccaggcaagggcctggagtgggtgtccaccatcagctaccaccaccacctgatcagccacgccgacagcgtgaagggcaggttcaccatcagcagggacaacagcaagaacaccctgtacctgcagatgaacagcctgagggccgaggacaccgccgtgtactactgcgcccgcatcaacaacgaccctatggatgtgtggggccagggcaccctggtgacagtgagctca

SEQ ID NO: 312 - protein, 117 aa, Homo sapiens
EVQLLESGGGLVQPGGSLRLSCAASGFTFSSYAMNWVRQAPGKGLEWVSTISYHHHLISHADSVKGRFTISRDNSKNTLYLQMNSLRAEDTAVYYCARINNDPMDVWGQGTLVTVSS

SEQ ID NO: 313 - protein, 5 aa, Homo sapiens
SYAMN

SEQ ID NO: 314 - protein, 17 aa, Homo sapiens
TISYHHHLISHADSVKG

SEQ ID NO: 315 - protein, 8 aa, Homo sapiens
INNDPMDV

SEQ ID NO: 316 - DNA, 333 bp, Homo sapiens; identical to SEQ ID NO: 16

SEQ ID NO: 317 - protein, 111 aa, Homo sapiens; identical to SEQ ID NO: 7

SEQ ID NO: 318 - protein, 11 aa, Homo sapiens
SGDNLGKKYVQ

SEQ ID NO: 319 - protein, 7 aa, Homo sapiens
DDSNRPS

SEQ ID NO: 320 - protein, 14 aa, Homo sapiens
QTWDGNPTTGETNV

SEQ ID NO: 321 - DNA, 351 bp, Homo sapiens
gaggtgcagctgctggagagcggcggagggctggtgcagccaggcggcagcctgaggctgtcctgcgccgcctccggattcaccttcagcagctacgccatgaactgggtgcggcaggccccaggcaagggcctggagtgggtgtccaccatcagctaccacgggcaccacatcagccacgccgaccaccataagggcaggttcaccatcagcagggacaacagcaagaacaccctgtacctgcagatgaacagcctgagggccgaggacaccgccgtgtactactgcgcccgcatcaacaacgaccctatggatgtgtggggccagggcaccctggtgacagtgagctca

SEQ ID NO: 322 - protein, 117 aa, Homo sapiens
EVQLLESGGGLVQPGGSLRLSCAASGFTFSSYAMNWVRQAPGKGLEWVSTISYHGHHISHADHHKGRFTISRDNSKNTLYLQMNSLRAEDTAVYYCARINNDPMDVWGQGTLVTVSS

SEQ ID NO: 323 - protein, 5 aa, Homo sapiens
SYAMN

SEQ ID NO: 324 - protein, 17 aa, Homo sapiens
TISYHGHHISHADHHKG

SEQ ID NO: 325 - protein, 8 aa, Homo sapiens
INNDPMDV

SEQ ID NO: 326 - DNA, 333 bp, Homo sapiens; identical to SEQ ID NO: 16

SEQ ID NO: 327 - protein, 111 aa, Homo sapiens; identical to SEQ ID NO: 7

SEQ ID NO: 328 - protein, 11 aa, Homo sapiens
SGDNLGKKYVQ

SEQ ID NO: 329 - protein, 7 aa, Homo sapiens
DDSNRPS

SEQ ID NO: 330 - protein, 14 aa, Homo sapiens
QTWDGNPTTGETNV

SEQ ID NO: 331 - DNA, 351 bp, Homo sapiens
gaggtgcagctgctggagagcggcggagggctggtgcagccaggcggcagcctgaggctgtcctgcgccgcctccggattcaccttcagcagctacgccatgaactgggtgcggcaggccccaggcaagggcctggagtgggtgtccaccatcagctaccacgggcaccacatcagctacgccgacagccatcatcacaggttcaccatcagcagggacaacagcaagaacaccctgtacctgcagatgaacagcctgagggccgaggacaccgccgtgtactactgcgcccgcatcaacaacgaccctatggatgtgtggggccagggcaccctggtgacagtgagctca

SEQ ID NO: 332 - protein, 117 aa, Homo sapiens
EVQLLESGGGLVQPGGSLRLSCAASGFTFSSYAMNWVRQAPGKGLEWVSTISYHGHHISYADSHHHRFTISRDNSKNTLYLQMNSLRAEDTAVYYCARINNDPMDVWGQGTLVTVSS

SEQ ID NO: 333 - protein, 5 aa, Homo sapiens
SYAMN

SEQ ID NO: 334 - protein, 17 aa, Homo sapiens
TISYHGHHISYADSHHH

SEQ ID NO: 335 - protein, 8 aa, Homo sapiens
INNDPMDV

SEQ ID NO: 336 - DNA, 333 bp, Homo sapiens; identical to SEQ ID NO: 16

SEQ ID NO: 337 - protein, 111 aa, Homo sapiens; identical to SEQ ID NO: 7

SEQ ID NO: 338 - protein, 11 aa, Homo sapiens
SGDNLGKKYVQ

SEQ ID NO: 339 - protein, 7 aa, Homo sapiens
DDSNRPS

SEQ ID NO: 340 - protein, 14 aa, Homo sapiens
QTWDGNPTTGETNV

SEQ ID NO: 341 - DNA, 351 bp, Homo sapiens
gaggtgcagctgctggagagcggcggagggctggtgcagccaggcggcagcctgaggctgtcctgcgccgcctccggattcaccttcagcagctacgccatgaactgggtgcggcaggccccaggcaagggcctggagtgggtgtccaccatccaccacagcgggcacctgcacagctaccaccaccacgtgaagggcaggttcaccatcagcagggacaacagcaagaacaccctgtacctgcagatgaacagcctgagggccgaggacaccgccgtgtactactgcgcccgcatcaacaacgaccctatggatgtgtggggccagggcaccctggtgacagtgagctca

SEQ ID NO: 342 - protein, 117 aa, Homo sapiens
EVQLLESGGGLVQPGGSLRLSCAASGFTFSSYAMNWVRQAPGKGLEWVSTIHHSGHLHSYHHHVKGRFTISRDNSKNTLYLQMNSLRAEDTAVYYCARINNDPMDVWGQGTLVTVSS

SEQ ID NO: 343 - protein, 5 aa, Homo sapiens
SYAMN

SEQ ID NO: 344 - protein, 17 aa, Homo sapiens
TIHHSGHLHSYHHHVKG

SEQ ID NO: 345 - protein, 8 aa, Homo sapiens
INNDPMDV

SEQ ID NO: 346 - DNA, 333 bp, Homo sapiens; identical to SEQ ID NO: 16

SEQ ID NO: 347 - protein, 111 aa, Homo sapiens; identical to SEQ ID NO: 7

SEQ ID NO: 348 - protein, 11 aa, Homo sapiens
SGDNLGKKYVQ

SEQ ID NO: 349 - protein, 7 aa, Homo sapiens
DDSNRPS

SEQ ID NO: 350 - protein, 14 aa, Homo sapiens
QTWDGNPTTGETNV

SEQ ID NO: 351 - DNA, 351 bp, Homo sapiens
gaggtgcagctgctggagagcggcggagggctggtgcagccaggcggcagcctgaggctgtcctgcgccgcctccggattcaccttcagcagctacgccatgaactgggtgcggcaggccccaggcaagggcctggagtgggtgtccaccatcagccacagcgggcacctgcaccactacgccgacagccataagcacaggttcaccatcagcagggacaacagcaagaacaccctgtacctgcagatgaacagcctgagggccgaggacaccgccgtgtactactgcgcccgcatcaacaacgaccctatggatgtgtggggccagggcaccctggtgacagtgagctca

SEQ ID NO: 352 - protein, 117 aa, Homo sapiens
EVQLLESGGGLVQPGGSLRLSCAASGFTFSSYAMNWVRQAPGKGLEWVSTISHSGHLHHYADSHKHRFTISRDNSKNTLYLQMNSLRAEDTAVYYCARINNDPMDVWGQGTLVTVSS

SEQ ID NO: 353 - protein, 5 aa, Homo sapiens
SYAMN

SEQ ID NO: 354 - protein, 17 aa, Homo sapiens
TISHSGHLHHYADSHKH

SEQ ID NO: 355 - protein, 8 aa, Homo sapiens
INNDPMDV

SEQ ID NO: 356 - DNA, 333 bp, Homo sapiens; identical to SEQ ID NO: 16

SEQ ID NO: 357 - protein, 111 aa, Homo sapiens; identical to SEQ ID NO: 7

SEQ ID NO: 358 - protein, 11 aa, Homo sapiens
SGDNLGKKYVQ

SEQ ID NO: 359 - protein, 7 aa, Homo sapiens
DDSNRPS

SEQ ID NO: 360 - protein, 14 aa, Homo sapiens
QTWDGNPTTGETNV

SEQ ID NO: 361 - DNA, 351 bp, Homo sapiens
gaggtgcagctgctggagagcggcggagggctggtgcagccaggcggcagcctgaggctgtcctgcgccgcctccggattcaccttcagcagctacgccatgaactgggtgcggcaggccccaggcaagggcctggagtgggtgtccaccatcagctaccacgggtcgcacatcagctaccacgacagcgtgcatcacaggttcaccatcagcagggacaacagcaagaacaccctgtacctgcagatgaacagcctgagggccgaggacaccgccgtgtactactgcgcccgcatcaacaacgaccctatggatgtgtggggccagggcaccctggtgacagtgagctca

SEQ ID NO: 362 - protein, 117 aa, Homo sapiens
EVQLLESGGGLVQPGGSLRLSCAASGFTFSSYAMNWVRQAPGKGLEWVSTISYHGSHISYHDSVHHRFTISRDNSKNTLYLQMNSLRAEDTAVYYCARINNDPMDVWGQGTLVTVSS

SEQ ID NO: 363 - protein, 5 aa, Homo sapiens
SYAMN

SEQ ID NO: 364 - protein, 17 aa, Homo sapiens
TISYHGSHISYHDSVHH

SEQ ID NO: 365 - protein, 8 aa, Homo sapiens
INNDPMDV

SEQ ID NO: 366 - DNA, 333 bp, Homo sapiens; identical to SEQ ID NO: 16

SEQ ID NO: 367 - protein, 111 aa, Homo sapiens; identical to SEQ ID NO: 7

SEQ ID NO: 368 - protein, 11 aa, Homo sapiens
SGDNLGKKYVQ

SEQ ID NO: 369 - protein, 7 aa, Homo sapiens
DDSNRPS

SEQ ID NO: 370 - protein, 14 aa, Homo sapiens
QTWDGNPTTGETNV

SEQ ID NO: 371 - DNA, 351 bp, Homo sapiens
gaggtgcagctgctggagagcggcggagggctggtgcagccaggcggcagcctgaggctgtcctgcgccgcctccggattcaccttcagcagctacgccatgaactgggtgcggcaggccccaggcaagggcctggagtgggtgtccaccatcagctaccacgggcaccacatcagccacgcccaccacgtgcatggcaggttcaccatcagcagggacaacagcaagaacaccctgtacctgcagatgaacagcctgagggccgaggacaccgccgtgtactactgcgcccgcatcaacaacgaccctatggatgtgtggggccagggcaccctggtgacagtgagctca

SEQ ID NO: 372 - protein, 117 aa, Homo sapiens
EVQLLESGGGLVQPGGSLRLSCAASGFTFSSYAMNWVRQAPGKGLEWVSTISYHGHHISHAHHVHGRFTISRDNSKNTLYLQMNSLRAEDTAVYYCARINNDPMDVWGQGTLVTVSS

SEQ ID NO: 373 - protein, 5 aa, Homo sapiens
SYAMN

SEQ ID NO: 374 - protein, 17 aa, Homo sapiens
TISYHGHHISHAHHVHG

SEQ ID NO: 375 - protein, 8 aa, Homo sapiens
INNDPMDV

SEQ ID NO: 376 - DNA, 333 bp, Homo sapiens; identical to SEQ ID NO: 16

SEQ ID NO: 377 - protein, 111 aa, Homo sapiens; identical to SEQ ID NO: 7

SEQ ID NO: 378 - protein, 11 aa, Homo sapiens
SGDNLGKKYVQ

SEQ ID NO: 379 - protein, 7 aa, Homo sapiens
DDSNRPS

SEQ ID NO: 380 - protein, 14 aa, Homo sapiens
QTWDGNPTTGETNV

SEQ ID NO: 381 - DNA, 351 bp, Homo sapiens
gaggtgcagctgctggagagcggcggagggctggtgcagccaggcggcagcctgaggctgtcctgcgccgcctccggattcaccttcagcagctacgccatgaactgggtgcggcaggccccaggcaagggcctggagtgggtgtccaccatcagctacagcgggtcgctgatcagctacgccgacagcgtgaagggcaggttcaccatcagcagggacaacagcaagaacaccctgtacctgcagatgaacagcctgagggccgaggacaccgccgtgtactactgcgcccgcatccaccaccaccctcacgatcactggggccagggcaccctggtgacagtgagctca

SEQ ID NO: 382 - protein, 117 aa, Homo sapiens
EVQLLESGGGLVQPGGSLRLSCAASGFTFSSYAMNWVRQAPGKGLEWVSTISYSGSLISYADSVKGRFTISRDNSKNTLYLQMNSLRAEDTAVYYCARIHHHPHDHWGQGTLVTVSS

SEQ ID NO: 383 - protein, 5 aa, Homo sapiens
SYAMN

SEQ ID NO: 384 - protein, 17 aa, Homo sapiens
TISYSGSLISYADSVKG

SEQ ID NO: 385 - protein, 8 aa, Homo sapiens
IHHHPHDH

SEQ ID NO: 386 - DNA, 333 bp, Homo sapiens; identical to SEQ ID NO: 16

SEQ ID NO: 387 - protein, 111 aa, Homo sapiens; identical to SEQ ID NO: 7

SEQ ID NO: 388 - protein, 11 aa, Homo sapiens
SGDNLGKKYVQ

SEQ ID NO: 389 - protein, 7 aa, Homo sapiens
DDSNRPS

SEQ ID NO: 390 - protein, 14 aa, Homo sapiens
QTWDGNPTTGETNV

SEQ ID NO: 391 - DNA, 351 bp, Homo sapiens
gaggtgcagctgctggagagcggcggagggctggtgcagccaggcggcagcctgaggctgtcctgcgccgcctccggattcaccttcagcagctacgccatgaactgggtgcggcaggccccaggcaagggcctggagtgggtgtccaccatcagctacagcgggtcgctgatcagctacgccgacagcgtgaagggcaggttcaccatcagcagggacaacagcaagaacaccctgtacctgcagatgaacagcctgagggccgaggacaccgccgtgtactactgcgcccgcatcaaccacgaccctatggatcactggggccagggcaccctggtgacagtgagctca

SEQ ID NO: 392 - protein, 117 aa, Homo sapiens
EVQLLESGGGLVQPGGSLRLSCAASGFTFSSYAMNWVRQAPGKGLEWVSTISYSGSLISYADSVKGRFTISRDNSKNTLYLQMNSLRAEDTAVYYCARINHDPMDHWGQGTLVTVSS

SEQ ID NO: 393 - protein, 5 aa, Homo sapiens
SYAMN

SEQ ID NO: 394 - protein, 17 aa, Homo sapiens
TISYSGSLISYADSVKG

SEQ ID NO: 395 - protein, 8 aa, Homo sapiens
INHDPMDH

SEQ ID NO: 396 - DNA, 333 bp, Homo sapiens; identical to SEQ ID NO: 16

SEQ ID NO: 397 - protein, 111 aa, Homo sapiens; identical to SEQ ID NO: 7

SEQ ID NO: 398 - protein, 11 aa, Homo sapiens
SGDNLGKKYVQ

SEQ ID NO: 399 - protein, 7 aa, Homo sapiens
DDSNRPS

SEQ ID NO: 400 - protein, 14 aa, Homo sapiens
QTWDGNPTTGETNV

SEQ ID NO: 401 - DNA, 351 bp, Homo sapiens; identical to SEQ ID NO: 71

SEQ ID NO: 402 - protein, 117 aa, Homo sapiens; identical to SEQ ID NO: 2

SEQ ID NO: 403 - protein, 5 aa, Homo sapiens
SYAMN

SEQ ID NO: 404 - protein, 17 aa, Homo sapiens
TISYSGSLISYADSVKG

SEQ ID NO: 405 - protein, 8 aa, Homo sapiens
INNDPMDV

SEQ ID NO: 406 - DNA, 333 bp, Homo sapiens
agtatcgagctgacccagccccccagcgtgagcgtgtccccaggccagaccgccagcatcacctgcagcggcgacaacctgggcaagaaatacgtgcagtggtatcagcagaagcccggccagtcccccgtgctggtgatctacgacgacagcaacaggcccagcggcatccccgagaggttcagcggcagcaacagcggcaacaccgccaccctgaccatcagcggcacccaggcgatggacgaggccgactactactgccacacctgggacgggcaccacacgacgggggagaccaaccacttcggcggagggaccaagttaaccgtccta

SEQ ID NO: 407 - protein, 111 aa, Homo sapiens
SIELTQPPSVSVSPGQTASITCSGDNLGKKYVQWYQQKPGQSPVLVIYDDSNRPSGIPERFSGSNSGNTATLTISGTQAMDEADYYCHTWDGHHTTGETNHFGGGTKLTVL

SEQ ID NO: 408 - protein, 11 aa, Homo sapiens
SGDNLGKKYVQ

SEQ ID NO: 409 - protein, 7 aa, Homo sapiens
DDSNRPS

SEQ ID NO: 410 - protein, 14 aa, Homo sapiens
HTWDGHHTTGETNH

SEQ ID NO: 411 - DNA, 351 bp, Homo sapiens; identical to SEQ ID NO: 71

SEQ ID NO: 412 - protein, 117 aa, Homo sapiens; identical to SEQ ID NO: 2

SEQ ID NO: 413 - protein, 5 aa, Homo sapiens
SYAMN

SEQ ID NO: 414 - protein, 17 aa, Homo sapiens
TISYSGSLISYADSVKG

SEQ ID NO: 415 - protein, 8 aa, Homo sapiens
INNDPMDV

SEQ ID NO: 416 - DNA, 333 bp, Homo sapiens
agtatcgagctgacccagccccccagcgtgagcgtgtccccaggccagaccgccagcatcacctgcagcggcgacaacctgggcaagaaatacgtgcagtggtatcagcagaagcccggccagtcccccgtgctggtgatctacgacgacagcaacaggcccagcggcatccccgagaggttcagcggcagcaacagcggcaacaccgccaccctgaccatcagcggcacccaggcgatggacgaggccgactactactgccagcactgggacgggcaccaccacacgggggagaccaacgtgttcggcggagggaccaagttaaccgtccta

SEQ ID NO: 417 - protein, 111 aa, Homo sapiens
SIELTQPPSVSVSPGQTASITCSGDNLGKKYVQWYQQKPGQSPVLVIYDDSNRPSGIPERFSGSNSGNTATLTISGTQAMDEADYYCQHWDGHHHTGETNVFGGGTKLTVL

SEQ ID NO: 418 - protein, 11 aa, Homo sapiens
SGDNLGKKYVQ

SEQ ID NO: 419 - protein, 7 aa, Homo sapiens
DDSNRPS

SEQ ID NO: 420 - protein, 14 aa, Homo sapiens
QHWDGHHHTGETNV

SEQ ID NO: 421 - DNA, 351 bp, Homo sapiens; identical to SEQ ID NO: 71

SEQ ID NO: 422 - protein, 117 aa, Homo sapiens; identical to SEQ ID NO: 2

SEQ ID NO: 423 - protein, 5 aa, Homo sapiens
SYAMN

SEQ ID NO: 424 - protein, 17 aa, Homo sapiens
TISYSGSLISYADSVKG

SEQ ID NO: 425 - protein, 8 aa, Homo sapiens
INNDPMDV

SEQ ID NO: 426 - DNA, 333 bp, Homo sapiens
agtatcgagctgacccagccccccagcgtgagcgtgtccccaggccagaccgccagcatcacctgcagcggcgacaacctgggcaagaaatacgtgcagtggtatcagcagaagcccggccagtcccccgtgctggtgatctacgacgacagcaacaggcccagcggcatccccgagaggttcagcggcagcaacagcggcaacaccgccaccctgaccatcagcggcacccaggcgatggacgaggccgactactactgccagcactggcacgggaacccgcacacgggggagcacaaccacttcggcggagggaccaagttaaccgtccta

SEQ ID NO: 427 - protein, 111 aa, Homo sapiens
SIELTQPPSVSVSPGQTASITCSGDNLGKKYVQWYQQKPGQSPVLVIYDDSNRPSGIPERFSGSNSGNTATLTISGTQAMDEADYYCQHWHGNPHTGEHNHFGGGTKLTVL

SEQ ID NO: 428 - protein, 11 aa, Homo sapiens
SGDNLGKKYVQ

SEQ ID NO: 429 - protein, 7 aa, Homo sapiens
DDSNRPS

SEQ ID NO: 430 - protein, 14 aa, Homo sapiens
QHWHGNPHTGEHNH

SEQ ID NO: 431 - DNA, 351 bp, Homo sapiens; identical to SEQ ID NO: 71

SEQ ID NO: 432 - protein, 117 aa, Homo sapiens; identical to SEQ ID NO: 2

SEQ ID NO: 433 - protein, 5 aa, Homo sapiens
SYAMN

SEQ ID NO: 434 - protein, 17 aa, Homo sapiens
TISYSGSLISYADSVKG

SEQ ID NO: 435 - protein, 8 aa, Homo sapiens
INNDPMDV

SEQ ID NO: 436 - DNA, 333 bp, Homo sapiens
agtatcgagctgacccagccccccagcgtgagcgtgtccccaggccagaccgccagcatcacctgcagcggcgacaacctgggcaagaaatacgtgcagtggtatcagcagaagcccggccagtcccccgtgctggtgatctacgacgacagcaacaggcccagcggcatccccgagaggttcagcggcagcaacagcggcaacaccgccaccctgaccatcagcggcacccaggcgatggacgaggccgactactactgccacacctgggaccacaacccgcaccatcatcacaccaaccacttcggcggagggaccaagttaaccgtccta

SEQ ID NO: 437 - protein, 111 aa, Homo sapiens
SIELTQPPSVSVSPGQTASITCSGDNLGKKYVQWYQQKPGQSPVLVIYDDSNRPSGIPERFSGSNSGNTATLTISGTQAMDEADYYCHTWDHNPHHHHTNHFGGGTKLTVL

SEQ ID NO: 438 - protein, 11 aa, Homo sapiens
SGDNLGKKYVQ

SEQ ID NO: 439 - protein, 7 aa, Homo sapiens
DDSNRPS

SEQ ID NO: 440 - protein, 14 aa, Homo sapiens
HTWDHNPHHHHTNH

SEQ ID NO: 441 - DNA, 351 bp, Homo sapiens; identical to SEQ ID NO: 71

SEQ ID NO: 442 - protein, 117 aa, Homo sapiens; identical to SEQ ID NO: 2

SEQ ID NO: 443 - protein, 5 aa, Homo sapiens
SYAMN

SEQ ID NO: 444 - protein, 17 aa, Homo sapiens
TISYSGSLISYADSVKG

SEQ ID NO: 445 - protein, 8 aa, Homo sapiens
INNDPMDV

SEQ ID NO: 446 - DNA, 333 bp, Homo sapiens
agtatcgagctgacccagccccccagcgtgagcgtgtccccaggccagaccgccagcatcacctgcagcggcgacaacctgggcaagaaatacgtgcagtggtatcagcagaagcccggccagtcccccgtgctggtgatctacgacgacagcaacaggcccagcggcatccccgagaggttcagcggcagcaacagcggcaacaccgccaccctgaccatcagcggcacccaggcgatggacgaggccgactactactgccaccactggcaccacaacccgacgcatcatgagaccaacgtgttcggcggagggaccaagttaaccgtccta

SEQ ID NO: 447 - protein, 111 aa, Homo sapiens
SIELTQPPSVSVSPGQTASITCSGDNLGKKYVQWYQQKPGQSPVLVIYDDSNRPSGIPERFSGSNSGNTATLTISGTQAMDEADYYCHHWHHNPTHHETNVFGGGTKLTVL

SEQ ID NO: 448 - protein, 11 aa, Homo sapiens
SGDNLGKKYVQ

SEQ ID NO: 449 - protein, 7 aa, Homo sapiens
DDSNRPS

SEQ ID NO: 450 - protein, 14 aa, Homo sapiens
HHWHHNPTHHETNV

SEQ ID NO: 451 - DNA, 351 bp, Homo sapiens; identical to SEQ ID NO: 71

SEQ ID NO: 452 - protein, 117 aa, Homo sapiens; identical to SEQ ID NO: 2

SEQ ID NO: 453 - protein, 5 aa, Homo sapiens
SYAMN

SEQ ID NO: 454 - protein, 17 aa, Homo sapiens
TISYSGSLISYADSVKG

SEQ ID NO: 455 - protein, 8 aa, Homo sapiens
INNDPMDV

SEQ ID NO: 456 - DNA, 333 bp, Homo sapiens
agtatcgagctgacccagccccccagcgtgagcgtgtccccaggccagaccgccagcatcacctgcagcggcgacaacctgggcaagaaatacgtgcagtggtatcagcagaagcccggccagtcccccgtgctggtgatctacgacgacagcaacaggcccagcggcatccccgagaggttcagcggcagcaacagcggcaacaccgccaccctgaccatcagcggcacccaggcgatggacgaggccgactactactgccagcactggcacgggcaccaccacacgggggagaccaacgtgttcggcggagggaccaagttaaccgtccta

SEQ ID NO: 457 - protein, 111 aa, Homo sapiens
SIELTQPPSVSVSPGQTASITCSGDNLGKKYVQWYQQKPGQSPVLVIYDDSNRPSGIPERFSGSNSGNTATLTISGTQAMDEADYYCQHWHGHHHTGETNVFGGGTKLTVL

SEQ ID NO: 458 - protein, 11 aa, Homo sapiens
SGDNLGKKYVQ

SEQ ID NO: 459 - protein, 7 aa, Homo sapiens
DDSNRPS

SEQ ID NO: 460 - protein, 14 aa, Homo sapiens
QHWHGHHHTGETNV

SEQ ID NO: 461 - DNA, 351 bp, Homo sapiens
gaggtgcagctgctcgagagcggcggagggctggtgcagccaggcggcagcctgaggctgtcctgcgccgcctccggattcaccttcagcagctacgccatgaactgggtgcggcaggccccaggcaagggcctggagtgggtgtccaccatcagctacagcgggtcgctgatccactacgccgacagcgtgaagggcaggttcaccatcagcagggacaacagcaagaacaccctgtacctgcagatgaacagcctgagggccgaggacaccgccgtgtactactgcgcccgcatcaaccacgaccctatggatgtgtggggccagggcaccctggtgacagtgagctca

SEQ ID NO: 462 - protein, 117 aa, Homo sapiens
EVQLLESGGGLVQPGGSLRLSCAASGFTFSSYAMNWVRQAPGKGLEWVSTISYSGSLIHYADSVKGRFTISRDNSKNTLYLQMNSLRAEDTAVYYCARINHDPMDVWGQGTLVTVSS

SEQ ID NO: 463 - protein, 5 aa, Homo sapiens
SYAMN

SEQ ID NO: 464 - protein, 17 aa, Homo sapiens
TISYSGSLIHYADSVKG

SEQ ID NO: 465 - protein, 8 aa, Homo sapiens
INHDPMDV

SEQ ID NO: 466 - DNA, 333 bp, Homo sapiens; identical to SEQ ID NO: 6

SEQ ID NO: 467 - protein, 111 aa, Homo sapiens; identical to SEQ ID NO: 7

SEQ ID NO: 468 - protein, 11 aa, Homo sapiens
SGDNLGKKYVQ

SEQ ID NO: 469 - protein, 7 aa, Homo sapiens
DDSNRPS

SEQ ID NO: 470 - protein, 14 aa, Homo sapiens
QTWDGNPTTGETNV

SEQ ID NO: 471 - DNA, 351 bp, Homo sapiens
gaggtgcagctgctggagagcggcggagggctggtgcagccaggcggcagcctgaggctgtcctgcgccgcctccggattcaccttcagcagctacgccatgaactgggtgcggcaggccccaggcaagggcctggagtgggtgtccaccatcagccacagcgggcaccacatcagccaccacgacagccatcatggcaggttcaccatcagcagggacaacagcaagaacaccctgtacctgcagatgaacagcctgagggccgaggacaccgccgtgtactactgcgcccgcatcaaccacgaccctatggatgtgtggggccagggcaccctggtgacagtgagctca

SEQ ID NO: 472 - protein, 117 aa, Homo sapiens
EVQLLESGGGLVQPGGSLRLSCAASGFTFSSYAMNWVRQAPGKGLEWVSTISHSGHHISHHDSHHGRFTISRDNSKNTLYLQMNSLRAEDTAVYYCARINHDPMDVWGQGTLVTVSS

SEQ ID NO: 473 - protein, 5 aa, Homo sapiens
SYAMN

SEQ ID NO: 474 - protein, 17 aa, Homo sapiens
TISHSGHHISHHDSHHG

SEQ ID NO: 475 - protein, 8 aa, Homo sapiens
INHDPMDV

SEQ ID NO: 476 - DNA, 333 bp, Homo sapiens; identical to SEQ ID NO: 16

SEQ ID NO: 477 - protein, 111 aa, Homo sapiens; identical to SEQ ID NO: 7

SEQ ID NO: 478 - protein, 11 aa, Homo sapiens
SGDNLGKKYVQ

SEQ ID NO: 479 - protein, 7 aa, Homo sapiens
DDSNRPS

SEQ ID NO: 480 - protein, 14 aa, Homo sapiens
QTWDGNPTTGETNV

SEQ ID NO: 481 - DNA, 351 bp, Homo sapiens
gaggtgcagctgctggagagcggcggagggctggtgcagccaggcggcagcctgaggctgtcctgcgccgcctccggattcaccttcagcagctacgccatgaactgggtgcggcaggccccaggcaagggcctggagtgggtgtccaccatcagccacagcgggcacctgatccaccacgccgacagccataagggcaggttcaccatcagcagggacaacagcaagaacaccctgtacctgcagatgaacagcctgagggccgaggacaccgccgtgtactactgcgcccgcatcaaccacgaccctatggatgtgtggggccagggcaccctggtgacagtgagctca

SEQ ID NO: 482 - protein, 117 aa, Homo sapiens
EVQLLESGGGLVQPGGSLRLSCAASGFTFSSYAMNWVRQAPGKGLEWVSTISHSGHLIHHADSHKGRFTISRDNSKNTLYLQMNSLRAEDTAVYYCARINHDPMDVWGQGTLVTVSS

SEQ ID NO: 483 - protein, 5 aa, Homo sapiens
SYAMN

SEQ ID NO: 484 - protein, 17 aa, Homo sapiens
TISHSGHLIHHADSHKG

SEQ ID NO: 485 - protein, 8 aa, Homo sapiens
INHDPMDV

SEQ ID NO: 486 - DNA, 333 bp, Homo sapiens; identical to SEQ ID NO: 16

SEQ ID NO: 487 - protein, 111 aa, Homo sapiens; identical to SEQ ID NO: 7

SEQ ID NO: 488 - protein, 11 aa, Homo sapiens
SGDNLGKKYVQ

SEQ ID NO: 489 - protein, 7 aa, Homo sapiens
DDSNRPS

SEQ ID NO: 490 - protein, 14 aa, Homo sapiens
QTWDGNPTTGETNV

SEQ ID NO: 491 - DNA, 351 bp, Homo sapiens
gaggtgcagctgctggagagcggcggagggctggtgcagccaggcggcagcctgaggctgtcctgcgccgcctccggattcaccttcagcagctacgccatgaactgggtgcggcaggccccaggcaagggcctggagtgggtgtccaccatcagctacagcgggcacctgatccactacgccgaccaccatcatggcaggttcaccatcagcagggacaacagcaagaacaccctgtacctgcagatgaacagcctgagggccgaggacaccgccgtgtactactgcgcccgcatcaaccacgaccctatggatgtgtggggccagggcaccctggtgacagtgagctca

SEQ ID NO: 492 - protein, 117 aa, Homo sapiens
EVQLLESGGGLVQPGGSLRLSCAASGFTFSSYAMNWVRQAPGKGLEWVSTISYSGHLIHYADHHHGRFTISRDNSKNTLYLQMNSLRAEDTAVYYCARINHDPMDVWGQGTLVTVSS

SEQ ID NO: 493 - protein, 5 aa, Homo sapiens
SYAMN

SEQ ID NO: 494 - protein, 17 aa, Homo sapiens
TISYSGHLIHYADHHHG

SEQ ID NO: 495 - protein, 8 aa, Homo sapiens
INHDPMDV

SEQ ID NO: 496 - DNA, 333 bp, Homo sapiens; identical to SEQ ID NO: 16

SEQ ID NO: 497 - protein, 111 aa, Homo sapiens; identical to SEQ ID NO: 7

SEQ ID NO: 498 - protein, 11 aa, Homo sapiens
SGDNLGKKYVQ

SEQ ID NO: 499 - protein, 7 aa, Homo sapiens
DDSNRPS

SEQ ID NO: 500 - protein, 14 aa, Homo sapiens
QTWDGNPTTGETNV

SEQ ID NO: 501 - DNA, 351 bp, Homo sapiens
gaggtgcagctgctggagagcggcggagggctggtgcagccaggcggcagcctgaggctgtcctgcgccgcctccggattcaccttcagcagctacgccatgaactgggtgcggcaggccccaggcaagggcctggagtgggtgtccaccatcagctaccacgggtcgcacatcagccacgccgaccacgtgcatggcaggttcaccatcagcagggacaacagcaagaacaccctgtacctgcagatgaacagcctgagggccgaggacaccgccgtgtactactgcgcccgcatcaaccacgaccctatggatgtgtggggccagggcaccctggtgacagtgagctca

SEQ ID NO: 502 - protein, 117 aa, Homo sapiens
EVQLLESGGGLVQPGGSLRLSCAASGFTFSSYAMNWVRQAPGKGLEWVSTISYHGSHISHADHVHGRFTISRDNSKNTLYLQMNSLRAEDTAVYYCARINHDPMDVWGQGTLVTVSS

SEQ ID NO: 503 - protein, 5 aa, Homo sapiens
SYAMN

SEQ ID NO: 504 - protein, 17 aa, Homo sapiens
TISYHGSHISHADHVHG

SEQ ID NO: 505 - protein, 8 aa, Homo sapiens
INHDPMDV

SEQ ID NO: 506 - DNA, 333 bp, Homo sapiens; identical to SEQ ID NO: 16

SEQ ID NO: 507 - protein, 111 aa, Homo sapiens; identical to SEQ ID NO: 7

SEQ ID NO: 508 - protein, 11 aa, Homo sapiens
SGDNLGKKYVQ

SEQ ID NO: 509 - protein, 7 aa, Homo sapiens
DDSNRPS

SEQ ID NO: 510 - protein, 14 aa, Homo sapiens
QTWDGNPTTGETNV

SEQ ID NO: 511 - DNA, 351 bp, Homo sapiens
gaggtgcagctgctggagagcggcggagggctggtgcagccaggcggcagcctgaggctgtcctgcgccgcctccggattcaccttcagcagctacgccatgaactgggtgcggcaggccccaggcaagggcctggagtgggtgtccaccatcagctaccacgggtcgcacatcagctaccacgacagccatcatggcaggttcaccatcagcagggacaacagcaagaacaccctgtacctgcagatgaacagcctgagggccgaggacaccgccgtgtactactgcgcccgcatcaaccacgaccctatggatgtgtggggccagggcaccctggtgacagtgagctca

SEQ ID NO: 512 - protein, 117 aa, Homo sapiens
EVQLLESGGGLVQPGGSLRLSCAASGFTFSSYAMNWVRQAPGKGLEWVSTISYHGSHISYHDSHHGRFTISRDNSKNTLYLQMNSLRAEDTAVYYCARINHDPMDVWGQGTLVTVSS

SEQ ID NO: 513 - protein, 5 aa, Homo sapiens
SYAMN

SEQ ID NO: 514 - protein, 17 aa, Homo sapiens
TISYHGSHISYHDSHHG

SEQ ID NO: 515 - protein, 8 aa, Homo sapiens
INHDPMDV

SEQ ID NO: 516 - DNA, 333 bp, Homo sapiens; identical to SEQ ID NO: 16

SEQ ID NO: 517 - protein, 111 aa, Homo sapiens; identical to SEQ ID NO: 7

SEQ ID NO: 518 - protein, 11 aa, Homo sapiens
SGDNLGKKYVQ

SEQ ID NO: 519 - protein, 7 aa, Homo sapiens
DDSNRPS

SEQ ID NO: 520 - protein, 14 aa, Homo sapiens
QTWDGNPTTGETNV

SEQ ID NO: 521 - DNA, 351 bp, Homo sapiens
gaggtgcagctgctggagagcggcggagggctggtgcagccaggcggcagcctgaggctgtcctgcgccgcctccggattcaccttcagcagctacgccatgaactgggtgcggcaggccccaggcaagggcctggagtgggtgtccaccatcagctaccacgggcaccacatcagctacgccgacagccatcatcacaggttcaccatcagcagggacaacagcaagaacaccctgtacctgcagatgaacagcctgagggccgaggacaccgccgtgtactactgcgcccgcatcaaccacgaccctatggatgtgtggggccagggcaccctggtgacagtgagctca

SEQ ID NO: 522 - protein, 117 aa, Homo sapiens
EVQLLESGGGLVQPGGSLRLSCAASGFTFSSYAMNWVRQAPGKGLEWVSTISYHGHHISYADSHHHRFTISRDNSKNTLYLQMNSLRAEDTAVYYCARINHDPMDVWGQGTLVTVSS

SEQ ID NO: 523 - protein, 5 aa, Homo sapiens
SYAMN

SEQ ID NO: 524 - protein, 17 aa, Homo sapiens
TISYHGHHISYADSHHH

SEQ ID NO: 525 - protein, 8 aa, Homo sapiens
INHDPMDV

SEQ ID NO: 526 - DNA, 333 bp, Homo sapiens; identical to SEQ ID NO: 16

SEQ ID NO: 527 - protein, 111 aa, Homo sapiens; identical to SEQ ID NO: 7

SEQ ID NO: 528 - protein, 11 aa, Homo sapiens
SGDNLGKKYVQ

SEQ ID NO: 529 - protein, 7 aa, Homo sapiens
DDSNRPS

SEQ ID NO: 530 - protein, 14 aa, Homo sapiens
QTWDGNPTTGETNV

SEQ ID NO: 531 - DNA, 351 bp, Homo sapiens
gaggtgcagctgctggagagcggcggagggctggtgcagccaggcggcagcctgaggctgtcctgcgccgcctccggattcaccttcagcagctacgccatgaactgggtgcggcaggccccaggcaagggcctggagtgggtgtccaccatcagctaccacgggtcgcacatcagctaccacgacagcgtgcatcacaggttcaccatcagcagggacaacagcaagaacaccctgtacctgcagatgaacagcctgagggccgaggacaccgccgtgtactactgcgcccgcatcaaccacgaccctatggatgtgtggggccagggcaccctggtgacagtgagctca

SEQ ID NO: 532 - protein, 117 aa, Homo sapiens
EVQLLESGGGLVQPGGSLRLSCAASGFTFSSYAMNWVRQAPGKGLEWVSTISYHGSHISYHDSVHHRFTISRDNSKNTLYLQMNSLRAEDTAVYYCARINHDPMDVWGQGTLVTVSS

SEQ ID NO: 533 - protein, 5 aa, Homo sapiens
SYAMN

SEQ ID NO: 534 - protein, 17 aa, Homo sapiens
TISYHGSHISYHDSVHH

SEQ ID NO: 535 - protein, 8 aa, Homo sapiens
INHDPMDV

SEQ ID NO: 536 - DNA, 333 bp, Homo sapiens; identical to SEQ ID NO: 16

SEQ ID NO: 537 - protein, 111 aa, Homo sapiens; identical to SEQ ID NO: 7

SEQ ID NO: 538 - protein, 11 aa, Homo sapiens
SGDNLGKKYVQ

SEQ ID NO: 539 - protein, 7 aa, Homo sapiens
DDSNRPS

SEQ ID NO: 540 - protein, 14 aa, Homo sapiens
QTWDGNPTTGETNV

SEQ ID NO: 541 - DNA, 351 bp, Homo sapiens
gaggtgcagctgctcgagagcggcggagggctggtgcagccaggcggcagcctgaggctgtcctgcgccgcctccggattcaccttcagcagctacgccatgaactgggtgcggcaggccccaggcaagggcctggagtgggtgtccaccatcagctacagcgggtcgctgatccactacgccgacagcgtgaagggcaggttcaccatcagcagggacaacagcaagaacaccctgtacctgcagatgaacagcctgagggccgaggacaccgccgtgtactactgcgcccgcatccaccacgaccctatggatgtgtggggccagggcaccctggtgacagtgagctca

SEQ ID NO: 542 - protein, 117 aa, Homo sapiens
EVQLLESGGGLVQPGGSLRLSCAASGFTFSSYAMNWVRQAPGKGLEWVSTISYSGSLIHYADSVKGRFTISRDNSKNTLYLQMNSLRAEDTAVYYCARIHHDPMDVWGQGTLVTVSS

SEQ ID NO: 543 - protein, 5 aa, Homo sapiens
SYAMN

SEQ ID NO: 544 - protein, 17 aa, Homo sapiens
TISYSGSLIHYADSVKG

SEQ ID NO: 545 - protein, 8 aa, Homo sapiens
IHHDPMDV

SEQ ID NO: 546 - DNA, 333 bp, Homo sapiens; identical to SEQ ID NO: 6

SEQ ID NO: 547 - protein, 111 aa, Homo sapiens; identical to SEQ ID NO: 7

SEQ ID NO: 548 - protein, 11 aa, Homo sapiens
SGDNLGKKYVQ

SEQ ID NO: 549 - protein, 7 aa, Homo sapiens
DDSNRPS

SEQ ID NO: 550 - protein, 14 aa, Homo sapiens
QTWDGNPTTGETNV

SEQ ID NO: 551 - DNA, 351 bp, Homo sapiens
gaggtgcagctgctggagagcggcggagggctggtgcagccaggcggcagcctgaggctgtcctgcgccgcctccggattcaccttcagcagctacgccatgaactgggtgcggcaggccccaggcaagggcctggagtgggtgtccaccatcagccacagcgggcaccacatcagccaccacgacagccatcatggcaggttcaccatcagcagggacaacagcaagaacaccctgtacctgcagatgaacagcctgagggccgaggacaccgccgtgtactactgcgcccgcatccaccacgaccctatggatgtgtggggccagggcaccctggtgacagtgagctca

SEQ ID NO: 552 - protein, 117 aa, Homo sapiens
EVQLLESGGGLVQPGGSLRLSCAASGFTFSSYAMNWVRQAPGKGLEWVSTISHSGHHISHHDSHHGRFTISRDNSKNTLYLQMNSLRAEDTAVYYCARIHHDPMDVWGQGTLVTVSS

SEQ ID NO: 553 - protein, 5 aa, Homo sapiens
SYAMN

SEQ ID NO: 554 - protein, 17 aa, Homo sapiens
TISHSGHHISHHDSHHG

SEQ ID NO: 555 - protein, 8 aa, Homo sapiens
IHHDPMDV

SEQ ID NO: 556 - DNA, 333 bp, Homo sapiens; identical to SEQ ID NO: 16

SEQ ID NO: 557 - protein, 111 aa, Homo sapiens; identical to SEQ ID NO: 7

SEQ ID NO: 558 - protein, 11 aa, Homo sapiens
SGDNLGKKYVQ

SEQ ID NO: 559 - protein, 7 aa, Homo sapiens
DDSNRPS

SEQ ID NO: 560 - protein, 14 aa, Homo sapiens
QTWDGNPTTGETNV

SEQ ID NO: 561 - DNA, 351 bp, Homo sapiens
gaggtgcagctgctggagagcggcggagggctggtgcagccaggcggcagcctgaggctgtcctgcgccgcctccggattcaccttcagcagctacgccatgaactgggtgcggcaggccccaggcaagggcctggagtgggtgtccaccatcagctacagcgggcacctgatccactacgccgaccaccatcatggcaggttcaccatcagcagggacaacagcaagaacaccctgtacctgcagatgaacagcctgagggccgaggacaccgccgtgtactactgcgcccgcatccaccacgaccctatggatgtgtggggccagggcaccctggtgacagtgagctca

SEQ ID NO: 562 - protein, 117 aa, Homo sapiens
EVQLLESGGGLVQPGGSLRLSCAASGFTFSSYAMNWVRQAPGKGLEWVSTISYSGHLIHYADHHHGRFTISRDNSKNTLYLQMNSLRAEDTAVYYCARIHHDPMDVWGQGTLVTVSS

SEQ ID NO: 563 - protein, 5 aa, Homo sapiens
SYAMN

SEQ ID NO: 564 - protein, 17 aa, Homo sapiens
TISYSGHLIHYADHHHG

SEQ ID NO: 565 - protein, 8 aa, Homo sapiens
IHHDPMDV

SEQ ID NO: 566 - DNA, 333 bp, Homo sapiens; identical to SEQ ID NO: 16

SEQ ID NO: 567 - protein, 111 aa, Homo sapiens; identical to SEQ ID NO: 7

SEQ ID NO: 568 - protein, 11 aa, Homo sapiens
SGDNLGKKYVQ

SEQ ID NO: 569 - protein, 7 aa, Homo sapiens
DDSNRPS

SEQ ID NO: 570 - protein, 14 aa, Homo sapiens
QTWDGNPTTGETNV

SEQ ID NO: 571 - DNA, 351 bp, Homo sapiens
gaggtgcagctgctggagagcggcggagggctggtgcagccaggcggcagcctgaggctgtcctgcgccgcctccggattcaccttcagcagctacgccatgaactgggtgcggcaggccccaggcaagggcctggagtgggtgtccaccatcagctaccacgggtcgcacatcagccacgccgaccacgtgcatggcaggttcaccatcagcagggacaacagcaagaacaccctgtacctgcagatgaacagcctgagggccgaggacaccgccgtgtactactgcgcccgcatccaccacgaccctatggatgtgtggggccagggcaccctggtgacagtgagctca

SEQ ID NO: 572 - protein, 117 aa, Homo sapiens
EVQLLESGGGLVQPGGSLRLSCAASGFTFSSYAMNWVRQAPGKGLEWVSTISYHGSHISHADHVHGRFTISRDNSKNTLYLQMNSLRAEDTAVYYCARIHHDPMDVWGQGTLVTVSS

SEQ ID NO: 573 - protein, 5 aa, Homo sapiens
SYAMN

SEQ ID NO: 574 - protein, 17 aa, Homo sapiens
TISYHGSHISHADHVHG

SEQ ID NO: 575 - protein, 8 aa, Homo sapiens
IHHDPMDV

SEQ ID NO: 576 - DNA, 333 bp, Homo sapiens; identical to SEQ ID NO: 16

SEQ ID NO: 577 - protein, 111 aa, Homo sapiens; identical to SEQ ID NO: 7

SEQ ID NO: 578 - protein, 11 aa, Homo sapiens
SGDNLGKKYVQ

SEQ ID NO: 579 - protein, 7 aa, Homo sapiens
DDSNRPS

SEQ ID NO: 580 - protein, 14 aa, Homo sapiens
QTWDGNPTTGETNV

SEQ ID NO: 581 - DNA, 351 bp, Homo sapiens
gaggtgcagctgctggagagcggcggagggctggtgcagccaggcggcagcctgaggctgtcctgcgccgcctccggattcaccttcagcagctacgccatgaactgggtgcggcaggccccaggcaagggcctggagtgggtgtccaccatcagctaccacgggtcgcacatcagctaccacgacagccatcatggcaggttcaccatcagcagggacaacagcaagaacaccctgtacctgcagatgaacagcctgagggccgaggacaccgccgtgtactactgcgcccgcatccaccacgaccctatggatgtgtggggccagggcaccctggtgacagtgagctca

SEQ ID NO: 582 - protein, 117 aa, Homo sapiens
EVQLLESGGGLVQPGGSLRLSCAASGFTFSSYAMNWVRQAPGKGLEWVSTISYHGSHISYHDSHHGRFTISRDNSKNTLYLQMNSLRAEDTAVYYCARIHHDPMDVWGQGTLVTVSS

SEQ ID NO: 583 - protein, 5 aa, Homo sapiens
SYAMN

SEQ ID NO: 584 - protein, 17 aa, Homo sapiens
TISYHGSHISYHDSHHG

SEQ ID NO: 585 - protein, 8 aa, Homo sapiens
IHHDPMDV

SEQ ID NO: 586 - DNA, 333 bp, Homo sapiens; identical to SEQ ID NO: 16

SEQ ID NO: 587 - protein, 111 aa, Homo sapiens; identical to SEQ ID NO: 7

SEQ ID NO: 588 - protein, 11 aa, Homo sapiens
SGDNLGKKYVQ

SEQ ID NO: 589 - protein, 7 aa, Homo sapiens
DDSNRPS

SEQ ID NO: 590 - protein, 14 aa, Homo sapiens
QTWDGNPTTGETNV

SEQ ID NO: 591 - DNA, 351 bp, Homo sapiens
gaggtgcagctgctggagagcggcggagggctggtgcagccaggcggcagcctgaggctgtcctgcgccgcctccggattcaccttcagcagctacgccatgaactgggtgcggcaggccccaggcaagggcctggagtgggtgtccaccatcagctaccacgggcaccacatcagctacgccgacagccatcatcacaggttcaccatcagcagggacaacagcaagaacaccctgtacctgcagatgaacagcctgagggccgaggacaccgccgtgtactactgcgcccgcatccaccacgaccctatggatgtgtggggccagggcaccctggtgacagtgagctca

SEQ ID NO: 592 - protein, 117 aa, Homo sapiens
EVQLLESGGGLVQPGGSLRLSCAASGFTFSSYAMNWVRQAPGKGLEWVSTISYHGHHISYADSHHHRFTISRDNSKNTLYLQMNSLRAEDTAVYYCARIHHDPMDVWGQGTLVTVSS

SEQ ID NO: 593 - protein, 5 aa, Homo sapiens
SYAMN

SEQ ID NO: 594 - protein, 17 aa, Homo sapiens
TISYHGHHISYADSHHH

SEQ ID NO: 595 - protein, 8 aa, Homo sapiens
IHHDPMDV

SEQ ID NO: 596 - DNA, 333 bp, Homo sapiens; identical to SEQ ID NO: 16

SEQ ID NO: 597 - protein, 111 aa, Homo sapiens; identical to SEQ ID NO: 7

SEQ ID NO: 598 - protein, 11 aa, Homo sapiens
SGDNLGKKYVQ

SEQ ID NO: 599 - protein, 7 aa, Homo sapiens
DDSNRPS

SEQ ID NO: 600 - protein, 14 aa, Homo sapiens
QTWDGNPTTGETNV

SEQ ID NO: 601 - DNA, 351 bp, Homo sapiens
gaggtgcagctgctggagagcggcggagggctggtgcagccaggcggcagcctgaggctgtcctgcgccgcctccggattcaccttcagcagctacgccatgaactgggtgcggcaggccccaggcaagggcctggagtgggtgtccaccatcagctaccacgggcaccacatcagctacgccgacagccatcatcacaggttcaccatcagcagggacaacagcaagaacaccctgtacctgcagatgaacagcctgagggccgaggacaccgccgtgtactactgcgcccgcatccaccacgaccctatggatcactggggccagggcaccctggtgacagtgagctca

SEQ ID NO: 602 - protein, 117 aa, Homo sapiens
EVQLLESGGGLVQPGGSLRLSCAASGFTFSSYAMNWVRQAPGKGLEWVSTISYHGHHISYADSHHHRFTISRDNSKNTLYLQMNSLRAEDTAVYYCARIHHDPMDHWGQGTLVTVSS

SEQ ID NO: 603 - protein, 5 aa, Homo sapiens
SYAMN

SEQ ID NO: 604 - protein, 17 aa, Homo sapiens
TISYHGHHISYADSHHH

SEQ ID NO: 605 - protein, 8 aa, Homo sapiens
IHHDPMDH

SEQ ID NO: 606 - DNA, 333 bp, Homo sapiens; identical to SEQ ID NO: 16

SEQ ID NO: 607 - protein, 111 aa, Homo sapiens; identical to SEQ ID NO: 7

SEQ ID NO: 608 - protein, 11 aa, Homo sapiens
SGDNLGKKYVQ

SEQ ID NO: 609 - protein, 7 aa, Homo sapiens
DDSNRPS

SEQ ID NO: 610 - protein, 14 aa, Homo sapiens
QTWDGNPTTGETNV

SEQ ID NO: 611 - DNA, 351 bp, Homo sapiens
gaggtgcagctgctggagagcggcggagggctggtgcagccaggcggcagcctgaggctgtcctgcgccgcctccggattcaccttcagcagctacgccatgaactgggtgcggcaggccccaggcaagggcctggagtgggtgtccaccatcagctaccacgggtcgcacatcagctaccacgacagcgtgcatcacaggttcaccatcagcagggacaacagcaagaacaccctgtacctgcagatgaacagcctgagggccgaggacaccgccgtgtactactgcgcccgcatccaccacgaccctatggatcactggggccagggcaccctggtgacagtgagctca

SEQ ID NO: 612 - protein, 117 aa, Homo sapiens
EVQLLESGGGLVQPGGSLRLSCAASGFTFSSYAMNWVRQAPGKGLEWVSTISYHGSHISYHDSVHHRFTISRDNSKNTLYLQMNSLRAEDTAVYYCARIHHDPMDHWGQGTLVTVSS

SEQ ID NO: 613 - protein, 5 aa, Homo sapiens
SYAMN

SEQ ID NO: 614 - protein, 17 aa, Homo sapiens
TISYHGSHISYHDSVHH

SEQ ID NO: 615 - protein, 8 aa, Homo sapiens
IHHDPMDH

SEQ ID NO: 616 - DNA, 333 bp, Homo sapiens; identical to SEQ ID NO: 16

SEQ ID NO: 617 - protein, 111 aa, Homo sapiens; identical to SEQ ID NO: 7

SEQ ID NO: 618 - protein, 11 aa, Homo sapiens
SGDNLGKKYVQ

SEQ ID NO: 619 - protein, 7 aa, Homo sapiens
DDSNRPS

SEQ ID NO: 620 - protein, 14 aa, Homo sapiens
QTWDGNPTTGETNV

SEQ ID NO: 621 - DNA, 351 bp, Homo sapiens
gaggtgcagctgctcgagagcggcggagggctggtgcagccaggcggcagcctgaggctgtcctgcgccgcctccggattcaccttcagcagctacgccatgaactgggtgcggcaggccccaggcaagggcctggagtgggtgtccaccatcagctacagcgggtcgctgatcagctacgccgacagcgtgaagggcaggttcaccatcagcagggacaacagcaagaacaccctgtacctgcagatgaacagcctgagggccgaggacaccgccgtgtactactgcgcccgcatcaaccacgaccctatggatgtgtggggccagggcaccctggtcaccgtctcctca

SEQ ID NO: 622 - protein, 117 aa, Homo sapiens; identical to SEQ ID NO: 32

SEQ ID NO: 623 - protein, 5 aa, Homo sapiens
SYAMN

SEQ ID NO: 624 - protein, 17 aa, Homo sapiens
TISYSGSLISYADSVKG

SEQ ID NO: 625 - protein, 8 aa, Homo sapiens
INHDPMDV

SEQ ID NO: 626 - DNA, 333 bp, Homo sapiens
agtatcgagctgacccagccccccagcgtgagcgtgtccccaggccagaccgccagcatcacctgcagcggcgacaacctgggcaagaaatacgtgcagtggtatcagcagaagcccggccagtcccccgtgctggtgatctacgacgacagcaacaggcccagcggcatccccgagaggttcagcggcagcaacagcggcaacaccgccaccctgaccatcagcggcacccaggccatggacgaggccgactactactgccagacctgggacgggaacccgacgcacggcgagaccaacgtgttcggcggagggaccaagctgaccgtccta

SEQ ID NO: 627 - protein, 111 aa, Homo sapiens; identical to SEQ ID NO: 47

SEQ ID NO: 628 - protein, 11 aa, Homo sapiens
SGDNLGKKYVQ

SEQ ID NO: 629 - protein, 7 aa, Homo sapiens
DDSNRPS

SEQ ID NO: 630 - protein, 14 aa, Homo sapiens
QTWDGNPTHGETNV

SEQ ID NO: 631 - DNA, 351 bp, Homo sapiens
gaggtgcagctgttggagagcggcggagggctggtgcagccaggcggcagcctgaggctgtcctgcgccgcctccggattcaccttcagcagctacgccatgaactgggtgcggcaggccccaggcaagggcctggagtgggtgtccaccatcagctacagcgggtcgctgatcagctacgccgacagcgtgaagggcaggttcaccatcagcagggacaacagcaagaacaccctgtacctgcagatgaacagcctgagggccgaggacaccgccgtgtactactgcgcccgcatccaccacgaccctatggatgtgtggggccagggcaccctggtcaccgtctcctca

SEQ ID NO: 632 - protein, 117 aa, Homo sapiens; identical to SEQ ID NO: 52

SEQ ID NO: 633 - protein, 5 aa, Homo sapiens
SYAMN

SEQ ID NO: 634 - protein, 17 aa, Homo sapiens
TISYSGSLISYADSVKG

SEQ ID NO: 635 - protein, 8 aa, Homo sapiens
IHHDPMDV

SEQ ID NO: 636 - DNA, 333 bp, Homo sapiens; identical to SEQ ID NO: 626

SEQ ID NO: 637 - protein, 111 aa, Homo sapiens; identical to SEQ ID NO: 47

SEQ ID NO: 638 - protein, 11 aa, Homo sapiens
SGDNLGKKYVQ

SEQ ID NO: 639 - protein, 7 aa, Homo sapiens
DDSNRPS

SEQ ID NO: 640 - protein, 14 aa, Homo sapiens
QTWDGNPTHGETNV

SEQ ID NO: 641 - DNA, 351 bp, Homo sapiens
gaggtgcagctgttggagagcggcggagggctggtgcagccaggcggcagcctgaggctgtcctgcgccgcctccggattcaccttcagcagctacgccatgaactgggtgcggcaggccccaggcaagggcctggagtgggtgtccaccatcagctaccacgggcaccacatcagctacgccgacagccatcatcacaggttcaccatcagcagggacaacagcaagaacaccctgtacctgcagatgaacagcctgagggccgaggacaccgccgtgtactactgcgcccgcatcaacaacgaccctatggatgtgtggggccagggcaccctggtcaccgtctcctca

SEQ ID NO: 642 - protein, 117 aa, Homo sapiens; identical to SEQ ID NO: 332

SEQ ID NO: 643 - protein, 5 aa, Homo sapiens
SYAMN

SEQ ID NO: 644 - protein, 17 aa, Homo sapiens
TISYHGHHISYADSHHH

SEQ ID NO: 645 - protein, 8 aa, Homo sapiens
INNDPMDV

SEQ ID NO: 646 - DNA, 333 bp, Homo sapiens; identical to SEQ ID NO: 626

SEQ ID NO: 647 - protein, 111 aa, Homo sapiens; identical to SEQ ID NO: 47

SEQ ID NO: 648 - protein, 11 aa, Homo sapiens
SGDNLGKKYVQ

SEQ ID NO: 649 - protein, 7 aa, Homo sapiens
DDSNRPS

SEQ ID NO: 650 - protein, 14 aa, Homo sapiens
QTWDGNPTHGETNV

SEQ ID NO: 651 - DNA, 351 bp, Homo sapiens
gaggtgcagctgctggagagcggcggagggctggtgcagccaggcggcagcctgaggctgtcctgcgccgcctccggattcaccttcagcagctacgccatgaactgggtgcggcaggccccaggcaagggcctggagtgggtgtccaccatcagctaccacgggcaccacatcagctacgccgacagccatcatcacaggttcaccatcagcagggacaacagcaagaacaccctgtacctgcagatgaacagcctgagggccgaggacaccgccgtgtactactgcgcccgcatcaaccacgaccctatggatgtgtggggccagggcaccctggtcaccgtctcctca

SEQ ID NO: 652 - protein, 117 aa, Homo sapiens; identical to SEQ ID NO: 522

SEQ ID NO: 653 - protein, 5 aa, Homo sapiens
SYAMN

SEQ ID NO: 654 - protein, 17 aa, Homo sapiens
TISYHGHHISYADSHHH

SEQ ID NO: 655 - protein, 8 aa, Homo sapiens
INHDPMDV

SEQ ID NO: 656 - DNA, 333 bp, Homo sapiens; identical to SEQ ID NO: 626

SEQ ID NO: 657 - protein, 111 aa, Homo sapiens; identical to SEQ ID NO: 47

SEQ ID NO: 658 - protein, 11 aa, Homo sapiens
SGDNLGKKYVQ

SEQ ID NO: 659 - protein, 7 aa, Homo sapiens
DDSNRPS

SEQ ID NO: 660 - protein, 14 aa, Homo sapiens
QTWDGNPTHGETNV

SEQ ID NO: 661 - DNA, 351 bp, Homo sapiens; identical to SEQ ID NO: 621

SEQ ID NO: 662 - protein, 117 aa, Homo sapiens; identical to SEQ ID NO: 32

SEQ ID NO: 663 - protein, 5 aa, Homo sapiens
SYAMN

SEQ ID NO: 664 - protein, 17 aa, Homo sapiens
TISYSGSLISYADSVKG

SEQ ID NO: 665 - protein, 8 aa, Homo sapiens
INHDPMDV

SEQ ID NO: 666 - DNA, 333 bp, Homo sapiens
agtatcgagctgacccagccccccagcgtgagcgtgtccccaggccagaccgccagcatcacctgcagcggcgacaacctgggcaagaaatacgtgcagtggtatcagcagaagcccggccagtcccccgtgctggtgatctacgacgacagcaacaggcccagcggcatccccgagaggttcagcggcagcaacagcggcaacaccgccaccctgaccatcagcggcacccaggcgatggacgaggccgactactactgccacacctggcaccaccacccgacgcatggggagcacaacgtgttcggcggagggaccaagctgaccgtccta

SEQ ID NO: 667 - protein, 111 aa, Homo sapiens; identical to SEQ ID NO: 97

SEQ ID NO: 668 - protein, 11 aa, Homo sapiens
SGDNLGKKYVQ

SEQ ID NO: 669 - protein, 7 aa, Homo sapiens
DDSNRPS

SEQ ID NO: 670 - protein, 14 aa, Homo sapiens
HTWHHHPTHGEHNV

SEQ ID NO: 671 - DNA, 351 bp, Homo sapiens; identical to SEQ ID NO: 641

SEQ ID NO: 672 - protein, 117 aa, Homo sapiens; identical to SEQ ID NO: 332

SEQ ID NO: 673 - protein, 5 aa, Homo sapiens
SYAMN

SEQ ID NO: 674 - protein, 17 aa, Homo sapiens
TISYHGHHISYADSHHH

SEQ ID NO: 675 - protein, 8 aa, Homo sapiens
INNDPMDV

SEQ ID NO: 676 - DNA, 333 bp, Homo sapiens; identical to SEQ ID NO: 666

SEQ ID NO: 677 - protein, 111 aa, Homo sapiens; identical to SEQ ID NO: 97

SEQ ID NO: 678 - protein, 11 aa, Homo sapiens
SGDNLGKKYVQ

SEQ ID NO: 679 - protein, 7 aa, Homo sapiens
DDSNRPS

SEQ ID NO: 680 - protein, 14 aa, Homo sapiens
HTWHHHPTHGEHNV

SEQ ID NO: 681 - DNA, 351 bp, Homo sapiens; identical to SEQ ID NO: 651

SEQ ID NO: 682 - protein, 117 aa, Homo sapiens; identical to SEQ ID NO: 522

SEQ ID NO: 683 - protein, 5 aa, Homo sapiens
SYAMN

SEQ ID NO: 684 - protein, 17 aa, Homo sapiens
TISYHGHHISYADSHHH

SEQ ID NO: 685 - protein, 8 aa, Homo sapiens
INHDPMDV

SEQ ID NO: 686 - DNA, 333 bp, Homo sapiens; identical to SEQ ID NO: 666

SEQ ID NO: 687 - protein, 111 aa, Homo sapiens; identical to SEQ ID NO: 97

SEQ ID NO: 688 - protein, 11 aa, Homo sapiens
SGDNLGKKYVQ

SEQ ID NO: 689 - protein, 7 aa, Homo sapiens
DDSNRPS

SEQ ID NO: 690 - protein, 14 aa, Homo sapiens
HTWHHHPTHGEHNV

SEQ ID NO: 691 - DNA, 351 bp, Homo sapiens; identical to SEQ ID NO: 621

SEQ ID NO: 692 - protein, 117 aa, Homo sapiens; identical to SEQ ID NO: 32

SEQ ID NO: 693 - protein, 5 aa, Homo sapiens
SYAMN

SEQ ID NO: 694 - protein, 17 aa, Homo sapiens
TISYSGSLISYADSVKG

SEQ ID NO: 695 - protein, 8 aa, Homo sapiens
INHDPMDV

SEQ ID NO: 696 - DNA, 333 bp, Homo sapiens
agtatcgagctgacccagccccccagcgtgagcgtgtccccaggccagaccgccagcatcacctgcagcggcgacaacctgggcaagaaatacgtgcagtggtatcagcagaagcccggccagtcccccgtgctggtgatctacgacgacagcaacaggcccagcggcatccccgagaggttcagcggcagcaacagcggcaacaccgccaccctgaccatcagcggcacccaggcgatggacgaggccgactactactgccacacctgggaccaccaccacacgacgggggagcacaacgtgttcggcggagggaccaagctgaccgtccta

SEQ ID NO: 697 - protein, 111 aa, Homo sapiens; identical to SEQ ID NO: 157

SEQ ID NO: 698 - protein, 11 aa, Homo sapiens
SGDNLGKKYVQ

SEQ ID NO: 699 - protein, 7 aa, Homo sapiens
DDSNRPS

SEQ ID NO: 700 - protein, 14 aa, Homo sapiens
HTWDHHHTTGEHNV

SEQ ID NO: 701 - DNA, 351 bp, Homo sapiens; identical to SEQ ID NO: 631

SEQ ID NO: 702 - protein, 117 aa, Homo sapiens; identical to SEQ ID NO: 52

SEQ ID NO: 703 - protein, 5 aa, Homo sapiens
SYAMN

SEQ ID NO: 704 - protein, 17 aa, Homo sapiens
TISYSGSLISYADSVKG

SEQ ID NO: 705 - protein, 8 aa, Homo sapiens
IHHDPMDV

SEQ ID NO: 706 - DNA, 333 bp, Homo sapiens; identical to SEQ ID NO: 696

SEQ ID NO: 707 - protein, 111 aa, Homo sapiens; identical to SEQ ID NO: 157

SEQ ID NO: 708 - protein, 11 aa, Homo sapiens
SGDNLGKKYVQ

SEQ ID NO: 709 - protein, 7 aa, Homo sapiens
DDSNRPS

SEQ ID NO: 710 - protein, 14 aa, Homo sapiens
HTWDHHHTTGEHNV

SEQ ID NO: 711 - DNA, 351 bp, Homo sapiens; identical to SEQ ID NO: 641

SEQ ID NO: 712 - protein, 117 aa, Homo sapiens; identical to SEQ ID NO: 332

SEQ ID NO: 713 - protein, 5 aa, Homo sapiens
SYAMN

SEQ ID NO: 714 - protein, 17 aa, Homo sapiens
TISYHGHHISYADSHHH

SEQ ID NO: 715 - protein, 8 aa, Homo sapiens
INNDPMDV

SEQ ID NO: 716 - DNA, 333 bp, Homo sapiens; identical to SEQ ID NO: 696

SEQ ID NO: 717 - protein, 111 aa, Homo sapiens; identical to SEQ ID NO: 157

SEQ ID NO: 718 - protein, 11 aa, Homo sapiens
SGDNLGKKYVQ

SEQ ID NO: 719 - protein, 7 aa, Homo sapiens
DDSNRPS

SEQ ID NO: 720 - protein, 14 aa, Homo sapiens
HTWDHHHTTGEHNV

SEQ ID NO: 721 - DNA, 351 bp, Homo sapiens; identical to SEQ ID NO: 621

SEQ ID NO: 722 - protein, 117 aa, Homo sapiens; identical to SEQ ID NO: 32

SEQ ID NO: 723 - protein, 5 aa, Homo sapiens
SYAMN

SEQ ID NO: 724 - protein, 17 aa, Homo sapiens
TISYSGSLISYADSVKG

SEQ ID NO: 725 - protein, 8 aa, Homo sapiens
INHDPMDV

SEQ ID NO: 726 - DNA, 333 bp, Homo sapiens
agtatcgagctgacccagccccccagcgtgagcgtgtccccaggccagaccgccagcatcacctgcagcggcgacaacctgggcaagaaatacgtgcagtggtatcagcagaagcccggccagtcccccgtgctggtgatctacgacgacagcaacaggcccagcggcatccccgagaggttcagcggcagcaacagcggcaacaccgccaccctgaccatcagcggcacccaggcgatggacgaggccgactactactgccagacctgggacgggcaccaccacacgggggagaccaaccacttcggcggagggaccaagctgaccgtccta

SEQ ID NO: 727 - protein, 111 aa, Homo sapiens; identical to SEQ ID NO: 197

SEQ ID NO: 728 - protein, 11 aa, Homo sapiens
SGDNLGKKYVQ

SEQ ID NO: 729 - protein, 7 aa, Homo sapiens
DDSNRPS

SEQ ID NO: 730 - protein, 14 aa, Homo sapiens
QTWDGHHHTGETNH

SEQ ID NO: 731 - DNA, 351 bp, Homo sapiens; identical to SEQ ID NO: 631

SEQ ID NO: 732 - protein, 117 aa, Homo sapiens; identical to SEQ ID NO: 52

SEQ ID NO: 733 - protein, 5 aa, Homo sapiens
SYAMN

SEQ ID NO: 734 - protein, 17 aa, Homo sapiens
TISYSGSLISYADSVKG

SEQ ID NO: 735 - protein, 8 aa, Homo sapiens
IHHDPMDV

SEQ ID NO: 736 - DNA, 333 bp, Homo sapiens; identical to SEQ ID NO: 726

SEQ ID NO: 737 - protein, 111 aa, Homo sapiens; identical to SEQ ID NO: 197

SEQ ID NO: 738 - protein, 11 aa, Homo sapiens
SGDNLGKKYVQ

SEQ ID NO: 739 - protein, 7 aa, Homo sapiens
DDSNRPS

SEQ ID NO: 740 - protein, 14 aa, Homo sapiens
QTWDGHHHTGETNH

SEQ ID NO: 741 - DNA, 351 bp, Homo sapiens; identical to SEQ ID NO: 641

SEQ ID NO: 742 - protein, 117 aa, Homo sapiens; identical to SEQ ID NO: 332

SEQ ID NO: 743 - protein, 5 aa, Homo sapiens
SYAMN

SEQ ID NO: 744 - protein, 17 aa, Homo sapiens
TISYHGHHISYADSHHH

SEQ ID NO: 745 - protein, 8 aa, Homo sapiens
INNDPMDV

SEQ ID NO: 746 - DNA, 333 bp, Homo sapiens; identical to SEQ ID NO: 726

SEQ ID NO: 747 - protein, 111 aa, Homo sapiens; identical to SEQ ID NO: 197

SEQ ID NO: 748 - protein, 11 aa, Homo sapiens
SGDNLGKKYVQ

SEQ ID NO: 749 - protein, 7 aa, Homo sapiens
DDSNRPS

SEQ ID NO: 750 - protein, 14 aa, Homo sapiens
QTWDGHHHTGETNH

SEQ ID NO: 751 - DNA, 351 bp, Homo sapiens; identical to SEQ ID NO: 651

SEQ ID NO: 752 - protein, 117 aa, Homo sapiens; identical to SEQ ID NO: 522

SEQ ID NO: 753 - protein, 5 aa, Homo sapiens
SYAMN

SEQ ID NO: 754 - protein, 17 aa, Homo sapiens
TISYHGHHISYADSHHH

SEQ ID NO: 755 - protein, 8 aa, Homo sapiens
INHDPMDV

SEQ ID NO: 756 - DNA, 333 bp, Homo sapiens; identical to SEQ ID NO: 726

SEQ ID NO: 757 - protein, 111 aa, Homo sapiens; identical to SEQ ID NO: 197

SEQ ID NO: 758 - protein, 11 aa, Homo sapiens
SGDNLGKKYVQ

SEQ ID NO: 759 - protein, 7 aa, Homo sapiens
DDSNRPS

SEQ ID NO: 760 - protein, 14 aa, Homo sapiens
QTWDGHHHTGETNH

SEQ ID NO: 761 - DNA, 351 bp, Homo sapiens; identical to SEQ ID NO: 621

SEQ ID NO: 762 - protein, 117 aa, Homo sapiens; identical to SEQ ID NO: 32

SEQ ID NO: 763 - protein, 5 aa, Homo sapiens
SYAMN

SEQ ID NO: 764 - protein, 17 aa, Homo sapiens
TISYSGSLISYADSVKG

SEQ ID NO: 765 - protein, 8 aa, Homo sapiens
INHDPMDV

SEQ ID NO: 766 - DNA, 333 bp, Homo sapiens
agtatcgagctgacccagccccccagcgtgagcgtgtccccaggccagaccgccagcatcacctgcagcggcgacaacctgggcaagaaatacgtgcagtggtatcagcagaagcccggccagtcccccgtgctggtgatctacgacgacagcaacaggcccagcggcatccccgagaggttcagcggcagcaacagcggcaacaccgccaccctgaccatcagcggcacccaggcgatggacgaggccgactactactgccacacctgggacgggcaccacacgacgggggagaccaaccacttcggcggagggaccaagctgaccgtccta

SEQ ID NO: 767 - protein, 111 aa, Homo sapiens; identical to SEQ ID NO: 407

SEQ ID NO: 768 - protein, 11 aa, Homo sapiens
SGDNLGKKYVQ

SEQ ID NO: 769 - protein, 7 aa, Homo sapiens
DDSNRPS

SEQ ID NO: 770 - protein, 14 aa, Homo sapiens
HTWDGHHTTGETNH

SEQ ID NO: 771 - DNA, 351 bp, Homo sapiens; identical to SEQ ID NO: 631

SEQ ID NO: 772 - protein, 117 aa, Homo sapiens; identical to SEQ ID NO: 52

SEQ ID NO: 773 - protein, 5 aa, Homo sapiens
SYAMN

SEQ ID NO: 774 - protein, 17 aa, Homo sapiens
TISYSGSLISYADSVKG

SEQ ID NO: 775 - protein, 8 aa, Homo sapiens
IHHDPMDV

SEQ ID NO: 776 - DNA, 333 bp, Homo sapiens; identical to SEQ ID NO: 766

SEQ ID NO: 777 - protein, 111 aa, Homo sapiens; identical to SEQ ID NO: 407

SEQ ID NO: 778 - protein, 11 aa, Homo sapiens
SGDNLGKKYVQ

SEQ ID NO: 779 - protein, 7 aa, Homo sapiens
DDSNRPS

SEQ ID NO: 780 - protein, 14 aa, Homo sapiens
HTWDGHHTTGETNH

SEQ ID NO: 781 - DNA, 351 bp, Homo sapiens; identical to SEQ ID NO: 641

SEQ ID NO: 782 - protein, 117 aa, Homo sapiens; identical to SEQ ID NO: 332

SEQ ID NO: 783 - protein, 5 aa, Homo sapiens
SYAMN

SEQ ID NO: 784 - protein, 17 aa, Homo sapiens
TISYHGHHISYADSHHH

SEQ ID NO: 785 - protein, 8 aa, Homo sapiens
INNDPMDV

SEQ ID NO: 786 - DNA, 333 bp, Homo sapiens; identical to SEQ ID NO: 766

SEQ ID NO: 787 - protein, 111 aa, Homo sapiens; identical to SEQ ID NO: 407

SEQ ID NO: 788 - protein, 11 aa, Homo sapiens
SGDNLGKKYVQ

SEQ ID NO: 789 - protein, 7 aa, Homo sapiens
DDSNRPS

SEQ ID NO: 790 - protein, 14 aa, Homo sapiens
HTWDGHHTTGETNH

SEQ ID NO: 791 - DNA, 351 bp, Homo sapiens; identical to SEQ ID NO: 651

SEQ ID NO: 792 - protein, 117 aa, Homo sapiens; identical to SEQ ID NO: 522

SEQ ID NO: 793 - protein, 5 aa, Homo sapiens
SYAMN

SEQ ID NO: 794 - protein, 17 aa, Homo sapiens
TISYHGHHISYADSHHH

SEQ ID NO: 795 - protein, 8 aa, Homo sapiens
INHDPMDV

SEQ ID NO: 796 - DNA, 333 bp, Homo sapiens; identical to SEQ ID NO: 766

SEQ ID NO: 797 - protein, 111 aa, Homo sapiens; identical to SEQ ID NO: 407

SEQ ID NO: 798 - protein, 11 aa, Homo sapiens
SGDNLGKKYVQ

SEQ ID NO: 799 - protein, 7 aa, Homo sapiens
DDSNRPS

SEQ ID NO: 800 - protein, 14 aa, Homo sapiens
HTWDGHHTTGETNH

SEQ ID NO: 801 - protein, 397 aa, Homo sapiens
MRSPSAAWLLGAAILLAASLSCSGTIQGTNRSSKGRSLIGKVDGTSHVTGKGVTVETVFSVDEFSASVLTGKLTTVFLPIVYTIVFVVGLPSNGMALWVFLFRTKKKHPAVIYMANLALADLLSVIWFPLKIAYHIHGNNWIYGEALCNVLIGFFYGNMYCSILFMTCLSVQRYWVIVNPMGHSRKKANIAIGISLAIWLLILLVTIPLYVVKQTIFIPALNITTCHDVLPEQLLVGDMFNYFLSLAIGVFLFPAFLTASAYVLMIRMLRSSAMDENSEKKRKRAIKLIVTVLAMYLICFTPSNLLLVVHYFLIKSQGQSHVYALYIVALCLSTLNSCIDPFVYYFVSHDFRDHAKNALLCRSVRTVKQMQVSLTSKKHSRKSSSYSSSSTTVKTSY

SEQ ID NO: 802 - protein, 39 aa, Homo sapiens
SLIGKVDGTSHVTGKGVTVETVFSVDEFSASVLTGKLTT

SEQ ID NO: 803 - protein, 30 aa, Homo sapiens
EVQLLESGGGLVQPGGSLRLSCAASGFTFS

SEQ ID NO: 804 - protein, 14 aa, Homo sapiens
WVRQAPGKGLEWVS

SEQ ID NO: 805 - protein, 32 aa, Homo sapiens
RFTISRDNSKNTLYLQMNSLRAEDTAVYYCAR

SEQ ID NO: 806 - protein, 11 aa, Homo sapiens
WGQGTLVTVSS

SEQ ID NO: 807 - protein, 22 aa, Homo sapiens
SIELTQPPSVSVSPGQTASITC

SEQ ID NO: 808 - protein, 15 aa, Homo sapiens
WYQQKPGQSPVLVIY

SEQ ID NO: 809 - protein, 32 aa, Homo sapiens
GIPERFSGSNSGNTATLTISGTQAMDEADYYC

SEQ ID NO: 810 - protein, 10 aa, Homo sapiens
FGGGTKLTVL

SEQ ID NO: 811 - protein, 17 aa, Homo sapiens
TISYSGSHISYHDSVHH

SEQ ID NO: 812 - protein, 17 aa, Homo sapiens
TISYHGSLISYHDSVHH

SEQ ID NO: 813 - protein, 17 aa, Homo sapiens
TISYHGSHISYADSVHH

SEQ ID NO: 814 - protein, 17 aa, Homo sapiens
TISYHGSHISYHDSVKH

SEQ ID NO: 815 - protein, 17 aa, Homo sapiens
TISYHGSHISYHDSVHG

SEQ ID NO: 816 - protein, 17 aa, Homo sapiens
TISYHGSLISYADSVKG

SEQ ID NO: 817 - protein, 17 aa, Homo sapiens
TISYSGSHISYADSVKG

SEQ ID NO: 818 - protein, 17 aa, Homo sapiens
TISYHGSHISYADSVKG

SEQ ID NO: 819 - protein, 8 aa, Homo sapiens
IHNDPMDV

SEQ ID NO: 820 - protein, 8 aa, Homo sapiens
INHDPMDV

SEQ ID NO: 821 - protein, 117 aa, Homo sapiens; identical to SEQ ID NO: 12

SEQ ID NO: 822 - protein, 117 aa, Homo sapiens
EVQLLESGGGLVQPGGSLRLSCAASGFTFSSYAMNWVRQAPGKGLEWVSTISYSGSHISYHDSVHHRFTISRDNSKNTLYLQMNSLRAEDTAVYYCARIHHDPMDVWGQGTLVTVSS

SEQ ID NO: 823 - protein, 117 aa, Homo sapiens
EVQLLESGGGLVQPGGSLRLSCAASGFTFSSYAMNWVRQAPGKGLEWVSTISYHGSLISYHDSVHHRFTISRDNSKNTLYLQMNSLRAEDTAVYYCARIHHDPMDVWGQGTLVTVSS

SEQ ID NO: 824 - protein, 117 aa, Homo sapiens
EVQLLESGGGLVQPGGSLRLSCAASGFTFSSYAMNWVRQAPGKGLEWVSTISYHGSHISYADSVHHRFTISRDNSKNTLYLQMNSLRAEDTAVYYCARIHHDPMDVWGQGTLVTVSS

SEQ ID NO: 825 - protein, 117 aa, Homo sapiens
EVQLLESGGGLVQPGGSLRLSCAASGFTFSSYAMNWVRQAPGKGLEWVSTISYHGSHISYHDSVKHRFTISRDNSKNTLYLQMNSLRAEDTAVYYCARIHHDPMDVWGQGTLVTVSS

SEQ ID NO: 826 - protein, 117 aa, Homo sapiens
EVQLLESGGGLVQPGGSLRLSCAASGFTFSSYAMNWVRQAPGKGLEWVSTISYHGSHISYHDSVHGRFTISRDNSKNTLYLQMNSLRAEDTAVYYCARIHHDPMDVWGQGTLVTVSS

SEQ ID NO: 827 - protein, 117 aa, Homo sapiens; identical to SEQ ID NO: 532

SEQ ID NO: 828 - protein, 117 aa, Homo sapiens
EVQLLESGGGLVQPGGSLRLSCAASGFTFSSYAMNWVRQAPGKGLEWVSTISYHGSHISYHDSVHHRFTISRDNSKNTLYLQMNSLRAEDTAVYYCARIHNDPMDVWGQGTLVTVSS

SEQ ID NO: 829 - protein, 117 aa, Homo sapiens
EVQLLESGGGLVQPGGSLRLSCAASGFTFSSYAMNWVRQAPGKGLEWVSTISYHGSLISYADSVKGRFTISRDNSKNTLYLQMNSLRAEDTAVYYCARIHHDPMDVWGQGTLVTVSS

SEQ ID NO: 830 - protein, 117 aa, Homo sapiens
EVQLLESGGGLVQPGGSLRLSCAASGFTFSSYAMNWVRQAPGKGLEWVSTISYSGSHISYADSVKGRFTISRDNSKNTLYLQMNSLRAEDTAVYYCARIHHDPMDVWGQGTLVTVSS

SEQ ID NO: 831 - protein, 117 aa, Homo sapiens
EVQLLESGGGLVQPGGSLRLSCAASGFTFSSYAMNWVRQAPGKGLEWVSTISYHGSHISYADSVKGRFTISRDNSKNTLYLQMNSLRAEDTAVYYCARIHHDPMDVWGQGTLVTVSS

SEQ ID NO: 832 - protein, 6 aa, Artificial Sequence
  source: /note="Description of Artificial Sequence: Synthetic peptide"
  MOD_RES (6)..(6): Ornithine
LIGRLX

SEQ ID NO: 833 - DNA, 351 bp, Homo sapiens
gaggtgcagctgctggagagcggcggagggctggtgcagccaggcggcagcctgaggctgtcctgcgccgcctccggattcaccttcagcagctacgccatgaactgggtgcggcaggccccaggcaagggcctggagtgggtgtccaccatcagctactccgggtcgcacatcagctaccacgacagcgtgcatcacaggttcaccatcagcagggacaacagcaagaacaccctgtacctgcagatgaacagcctgagggccgaggacaccgccgtgtactactgcgcccgcatccaccacgaccctatggatgtgtggggccagggcaccctggtgacagtgagctca

SEQ ID NO: 834 - DNA, 351 bp, Homo sapiens
gaggtgcagctgctggagagcggcggagggctggtgcagccaggcggcagcctgaggctgtcctgcgccgcctccggattcaccttcagcagctacgccatgaactgggtgcggcaggccccaggcaagggcctggagtgggtgtccaccatcagctaccacgggtcgctcatcagctaccacgacagcgtgcatcacaggttcaccatcagcagggacaacagcaagaacaccctgtacctgcagatgaacagcctgagggccgaggacaccgccgtgtactactgcgcccgcatccaccacgaccctatggatgtgtggggccagggcaccctggtgacagtgagctca

SEQ ID NO: 835 - DNA, 351 bp, Homo sapiens
gaggtgcagctgctggagagcggcggagggctggtgcagccaggcggcagcctgaggctgtcctgcgccgcctccggattcaccttcagcagctacgccatgaactgggtgcggcaggccccaggcaagggcctggagtgggtgtccaccatcagctaccacgggtcgcacatcagctacgccgacagcgtgcatcacaggttcaccatcagcagggacaacagcaagaacaccctgtacctgcagatgaacagcctgagggccgaggacaccgccgtgtactactgcgcccgcatccaccacgaccctatggatgtgtggggccagggcaccctggtgacagtgagctca

SEQ ID NO: 836 - DNA, 351 bp, Homo sapiens
gaggtgcagctgctggagagcggcggagggctggtgcagccaggcggcagcctgaggctgtcctgcgccgcctccggattcaccttcagcagctacgccatgaactgggtgcggcaggccccaggcaagggcctggagtgggtgtccaccatcagctaccacgggtcgcacatcagctaccacgacagcgtgaagcacaggttcaccatcagcagggacaacagcaagaacaccctgtacctgcagatgaacagcctgagggccgaggacaccgccgtgtactactgcgcccgcatccaccacgaccctatggatgtgtggggccagggcaccctggtgacagtgagctca

SEQ ID NO: 837 - DNA, 351 bp, Homo sapiens
gaggtgcagctgctggagagcggcggagggctggtgcagccaggcggcagcctgaggctgtcctgcgccgcctccggattcaccttcagcagctacgccatgaactgggtgcggcaggccccaggcaagggcctggagtgggtgtccaccatcagctaccacgggtcgcacatcagctaccacgacagcgtgcatggcaggttcaccatcagcagggacaacagcaagaacaccctgtacctgcagatgaacagcctgagggccgaggacaccgccgtgtactactgcgcccgcatccaccacgaccctatggatgtgtggggccagggcaccctggtgacagtgagctca

SEQ ID NO: 838 - DNA, 351 bp, Homo sapiens
gaggtgcagctgctggagagcggcggagggctggtgcagccaggcggcagcctgaggctgtcctgcgccgcctccggattcaccttcagcagctacgccatgaactgggtgcggcaggccccaggcaagggcctggagtgggtgtccaccatcagctaccacgggtcgcacatcagctaccacgacagcgtgcatcacaggttcaccatcagcagggacaacagcaagaacaccctgtacctgcagatgaacagcctgagggccgaggacaccgccgtgtactactgcgcccgcatccacaacgaccctatggatgtgtggggccagggcaccctggtgacagtgagctca

SEQ ID NO: 839 - DNA, 351 bp, Homo sapiens
gaggtgcagctgctggagagcggcggagggctggtgcagccaggcggcagcctgaggctgtcctgcgccgcctccggattcaccttcagcagctacgccatgaactgggtgcggcaggccccaggcaagggcctggagtgggtgtccaccatcagctaccacgggtcgctcatcagctacgccgacagcgtgaagggcaggttcaccatcagcagggacaacagcaagaacaccctgtacctgcagatgaacagcctgagggccgaggacaccgccgtgtactactgcgcccgcatccaccacgaccctatggatgtgtggggccagggcaccctggtgacagtgagctca

SEQ ID NO: 840 - DNA, 351 bp, Homo sapiens
gaggtgcagctgctggagagcggcggagggctggtgcagccaggcggcagcctgaggctgtcctgcgccgcctccggattcaccttcagcagctacgccatgaactgggtgcggcaggccccaggcaagggcctggagtgggtgtccaccatcagctactccgggtcgcacatcagctacgccgacagcgtgaagggcaggttcaccatcagcagggacaacagcaagaacaccctgtacctgcagatgaacagcctgagggccgaggacaccgccgtgtactactgcgcccgcatccaccacgaccctatggatgtgtggggccagggcaccctggtgacagtgagctca

SEQ ID NO: 841 - DNA, 351 bp, Homo sapiens
gaggtgcagctgctggagagcggcggagggctggtgcagccaggcggcagcctgaggctgtcctgcgccgcctccggattcaccttcagcagctacgccatgaactgggtgcggcaggccccaggcaagggcctggagtgggtgtccaccatcagctaccacgggtcgcacatcagctacgccgacagcgtgaagggcaggttcaccatcagcagggacaacagcaagaacaccctgtacctgcagatgaacagcctgagggccgaggacaccgccgtgtactactgcgcccgcatccaccacgaccctatggatgtgtggggccagggcaccctggtgacagtgagctca